European Patent Application EP 4 389 874 A1, published June 26, 2024. Title: Genetically modified microorganisms for the manufacture of compounds derived from dihydroxyacetone phosphate. Applicant: Acies Bio D O O. The sequence listing filed with the application follows.

SEQUENCE LISTING (214 sequences)

SEQ ID NO: 1 - protein, 381 aa, synthetic construct
MTNFFIPPASVIGRGAVKEVGTRLKQIGAKKALIVTDAFLHSTGLSEEVAKNIREAGLDVAIFPKAQPDPADTQVHEGVDVFKQENCDALVSIGGGSSHDTAKAIGLVAANGGRINDYQGVNSVEKPVVPVVAITTTAGTGSETTSLAVITDSARKVKMPVIDEKITPTVAIVDPELMVKKPAGLTIATGMDALSHAIEAYVAKGATPVTDAFAIQAMKLINEYLPKAVANGEDIEAREAMAYAQYMAGVAFNNGGLGLVHSISHQVGGVYKLQHGICNSVNMPHVCAFNLIAKTERFAHIAELLGENVSGLSTAAAAERAIVALERYNKNFGIPSGYAEMGVKEEDIELLAKNAFEDVCTQSNPRVATVQDIAQIIKNAL

SEQ ID NO: 2 - protein, 1225 aa, synthetic construct
MVYVARGAARETLDRPQMKQALFAALDALGPRAKVLVLPPDFTRFHSQAGILTQYVWEYYGDRLAAVLPALGTHSPMTEAQLREMFGAMPLHLFKPHDWRNDVVTLGTVPPEYVRELTEGRLDFEWPVQVNKLLVEGGFDLILSIGQVVPHEVIGMANYNKNLFVGTGGAVAINRSHFVGAVYGMERIMGRADTPVRRLFNYGSDHFGHLLPQTVYVQTVVGRADDGGMAVRGLYVGDDIEVFNRAAALALEVNFEMVPKPFKKCVVYLDPSEFKSTWLGNKAVYRTRMAMADGGELLILAPGVKEFGEDAQIDALIRKYGYFGTPRTLEAVRANADLQENLGAAAHLIHGSSEGRFTITYAPGHLSRAEIDRLGIRAIIVEGAPPEGKLFGLKIHREGVEFLHLDEYRGWKNYELNEALRQKHGKKISAATIGIAGERRYKSASVSFSDMMGDPSRNAARGGLGSVMAAKGLKAIVIDASGAAPVDIAKKEFFREAVKSWVETINKDVTCWLFRQFGTPLAVSTNSYQGTMPWQNYTSGRPEGFQKVSGETIKKLNLERGGRMHGCMPGCVIQCSILYNNPDGTRLCAAQEYEALGLLGTNLGITDPDAIGRMKYLCDDIGIDLIEIGCALGVAAQGGKLKMGDAEGAIGLLQEVEKGSAFGKVLGDGVVATARDLGISRVPAFKGQGIPAHDGRAVKGIGVTYATSPMGADHTAGLTYRLTLSKTGQAANSLRFQVAASACDTFGYCLNAVPGGSASLYSFLADLLAARYGSNVSGEDVLRIAKETLKDERKFNAAAGFEKIWEKVPSFYRNEPLPPTNSVFDVDDAEIERIWDGLDAFKEPKQLWEMRFDPMPPLLFGTGVIRLLGERTKQLKIKKALLIADPIMGKLGTTGEIQRILEKSGIASAVFSDVEPDPPVEEIEKIGQLYRQEKCDGLIALGGGSSMDAGKAAAIRVSQSGPMTEFEAAMGGGGKIKPPMPPLICIPTTSGTGSEVNTYAIITDRERSKKFLIISRYIIPSLAVIDPNITRTMPKGLTAETGVDALAHCIEGYVSKITPFHPYYAGLGLAGVKLIGNSLRKACSNPDDMNARMEMCMAAIDGGIAFSKGLGLGHAIGHAVGAQYHVSHGKSLAVSLLCFVRVNREVCKEEFRDLALVLDRTEDLEKALERLYRDVNLPTRFRDLGIPEGGLKSLAFEVGKDAANLAGNPVPMSDRKILEILKEFY

SEQ ID NO: 3 - protein, 385 aa, synthetic construct
MSHFQFQTVPNIISGLGSIQELQNVLASKTYRKLLLVTDAGMIKNQLHLPILQILDTLKIEHVIYADVQADPPEQVVLDAANYAKQQNVDVIVGFGGGSSLDVAKVIALLAHPNQTQNLQEMYGVNQVKTTRLPLILIPTTAGTGSEVTPISIVTTGETTKMGIVSPVLYADTAILDATFTQNLPAHITAATGIDAMVHAIEAYTSKHKKNIYTDILAKHALKLLNHNLPKVLKNGNDLEARQNMLFGSMLAGQAFANSPVAAVHALAYPLGGHFHLSHGHTNALVLVEVLKFNAPYAKQYYAELMQWLDPYSNGSTDGLCDLFIDHMQNHLDRSGLTLKLSDLSIEESSLPRLAQDAMLQTRLLQNNPRDMTEAAALAIYQAIY

SEQ ID NO: 4 - protein, 573 aa, synthetic construct
MADADLDKQVNTAGAWPIATGGYYSQHNSPLAQINKSNVKNVKAAWSFSTGVLNGHEGAPLVIGDMMYVHSAFPNNTYALNLNDPGKIVWQHKPKQDASTKAVMCCDVVDRGLAYGAGQIVKKQANGHLLALDAKTGKINWEVEVCDPKVGSTLTQAPFVAKDTVLMGCSGAELGVRGAVNAFDLKTGELKWRAFATGSDDSVRLAKDFNSANPHYGQFGLGTKTWEGDAWKIGGGTNWGWYAYDPKLNLFYYGSGNPAPWNETMRPGDNKWTMTIWGRDLDTGMAKWGYQKTPHDEWDFAGVNQMVLTDQPVNGKMTPLLSHIDRNGILYTLNRENGNLIVAEKVDPAVNVFKKVDLKTGTPVRDPEFATRMDHKGTNICPSAMGFHNQGVDSYDPESRTLYAGLNHICMDWEPFMLPYRAGQFFVGATLAMYPGPNGPTKKEMGQIRAFDLTTGKAKWTKWEKFAAWGGTLYTKGGLVWYATLDGYLKALDNKDGKELWNFKMPSGGIGSPMTYSFKGKQYIGSMYGVGGWPGVGLVFDLTDPSAGLGAVGAFRELQNHTQMGGGLMVFSL

SEQ ID NO: 5 - protein, 626 aa, synthetic construct
MSRFVTSVSALAMLALAPAALSSGAYANDKLVELSKSDDNWVMPGKNYDSNNFSDLKQINKGNVKQLRPAWTFSTGLLNGHEGAPLVVDGKMYIHTSFPNNTFALGLDDPGTILWQDKPKQNPAARAVACCDLVNRGLAYWPGDGKTPALILKTQLDGNVAALNAETGETVWKVENSDIKVGSTLTIAPYVVKDKVIIGSSGAELGVRGYLTAYDVKTGEQVWRAYATGPDKDLLLASDFNIKNPHYGQKGLGTGTWEGDAWKIGGGTNWGWYAYDPGTNLIYFGTGNPAPWNETMRPGDNKWTMTIFGRDADTGEAKFGYQKTPHDEWDYAGVNVMMLSEQKDKDGKARKLLTHPDRNGIVYTLDRTDGALVSANKLDDTVNVFKSVDLKTGQPVRDPEYGTRMDHLAKDICPSAMGYHNQGHDSYDPKRELFFMGINHICMDWEPFMLPYRAGQFFVGATLNMYPGPKGDRQNYEGLGQIKAYNAITGDYKWEKMERFAVWGGTMATAGDLVFYGTLDGYLKARDSDTGDLLWKFKIPSGAIGYPMTYTHKGTQYVAIYYGVGGWPGVGLVFDLADPTAGLGAVGAFKKLANYTQMGGGVVVFSLDGKGPYDDPNVGEWKSAAK

SEQ ID NO: 6 - protein, 181 aa, synthetic construct
NWGWYAYDPKLNLFYYGSGNPAPWNETMRPGDNKWTMTIWARDLDTGEAKWGYQKTPHDEWDFAGVNQMILSDHKVDGKVTPLLTHIDRNGIMYTLNRDNGNLIQAAKVDPAVNVFKKVDLKTGTPVRDPEFSTRMDHKSTNVCPSAMGFHNQGLDALDLDEPIVYAGLNHICMDWEPFML

SEQ ID NO: 7 - protein, 618 aa, synthetic construct
MKKPLKSLLLASSVAALLATPVISSANSGVEKLTKNPANWATALGNYSGTRYSKLDQINSKNVKNLQPAWSFSTGVLRGHEGGPLVIGDVIYIHTPFPNTVYALDQATRSVIWEYTPTMDADVTIPVMCCDTVNRGLAYGDGKIFLQQSDTVLTALDAKTGQRIWSVQNGDPKLGMTNTQAPLVVNDKVITGIAGGEFGVRGFLAAYDIKTGELSWKGYSMGPDGDTLIKPGSSTTWENGKVTKLGKNSGTSSWEGDQWKIGGGTTWGWYSYDPDLNLIYYGSGNPSTWNPVQRPGDNKWSMSLWARDADTGEVKWVYQMTPHDEWDFDGINEVVLADQKIGGKTRKTVVHFDRNGFGYTLDRVTGELLVAEKFDKTVNWASHVDLKSGRPQVVSEFSTEQNGEDENTEGVCPAALGSKNQQPVSYSPKTKMFYISANHLCMDYEPFEVSYTAGQPYVGATLTMMPAGGDVLTGKKDGSTNLGQFTAWDATTGKIVWSNKETFSVWSGSVATAGDVVFYGTLEGYLKAVDAKTGKELYKFKTPSGIIGNVNTWSYKGKQYVGVLSGIGGWAGIGIAAGLDSGESDSNSEGLGAVGAYRSLSSFTKLGGVFTVFSLPGK

SEQ ID NO: 8 - protein, 399 aa, synthetic construct
MSGNRGVVYLGSGKVEVQKIDYPKMQDPRGKKIEHGVILKVVSTNICGSDQHMVRGRTTAQVGLVLGHEITGEVIEKGRDVENLQIGDLVSVPFNVACGRCRSCKEMHTGVCLTVNPARAGGAYGYVDMGDWTGGQAEYLLVPYADFNLLKLPDRDKAMEKIRDLTCLSDILPTGYHGAVTAGVGPGSTVYVAGAGPVGLAAAASARLLGAAVVIVGDLNPARLAHAKAQGFEIADLSLDTPLHEQIAALLGEPEVDCAVDAVGFEARGHGHEGAKHEAPATVLNSLMQVTRVAGKIGIPGLYVTEDPGAVDAAAKIGSLSIRFGLGWAKSHSFHTGQTPVMKYNRALMQAIMWDRINIAEVVGVQVISLDDAPRGYGEFDAGVPKKFVIDPHKTFSAA

SEQ ID NO: 9 - protein, 402 aa, synthetic construct
MKAVVFHGIGDIRIDTVPDPGLAQTTDAVVRLTSSAICGTDLHMVRGTLGGMKPGTILGHEGVGLVEEVGRDVRNLRRGDRVLIPSTISCGHCAYCRAGYTAQCDTANPGGPLAGTAFFGGPQASGAFDGLQAEYARTPFAHASLIRLPDSLDDERAILMSDIFPTGYFGAQLAEVRMGDTVAVFGAGPVGQFAIASAKLMGAGRVIAIDRVVSRLEMACAQGAEVINFDDDDPVDTILQLTGGIGVDRVIDAVGVDAVRPTRGPAAPHDAQSRRAFDDEVRELAPRTRADGGHWVPGDAPSQVLQWAVRAVAKAGTVSIIGVYPMNDRFFPIGAAMNRNLTVKMGNCNHRAITPKLIEIVRSGAFDPITVLTQAEPLTSAIDAYRAFDTREPGWIKVKLEP

SEQ ID NO: 10 - protein, 390 aa, synthetic construct
MRALTYHGSKDVRIETVPDPVLQADDDIIIRVTSTAICGSDLHLYRGKIPQLHDGDILGHEFMGIVEDTGHGVTEVRKGDRVIIPFVIACGHCFFCAQQQFAACETTNPGPGPSLNKKSGTPPAALFGYSHLYGGIPGGQAELVRVPHGNVGPFKINGSLADEQVLFLTDILPTGYQAVLNAGVGKGSSLAIFGAGPVGLMAAACARMMGVETIFMIDDLQYRLDFAQAQYNTISINLDEVEDPADYILEHTAHRGVDGSIDAVGFEAKGSVVESALTALKLETSNGKVIRQCIAATRRGGTVSIPGVYAGFIHGFLIGDAFDKGLTFKMGQTHVHRFLPELLEFIENGDLHPADIITHRMALEDAPLGYRIFNDAEENCRKVVLTPGLH

SEQ ID NO: 11 - protein, 396 aa, synthetic construct
MASQSMKALNYVGPFTVQVQEVERPKLEHPDDIIVKVTSAAICGSDLHMYEGRTAAEPGITFGHENLGLVEELGEGVTLLKKGDRVVMPFNVADGRCRNCEEGKTAFCTGVNPGFAGGAYGYVAMGPCRGGQAQYLRVPYADFNALKLPPGTEHEADFILLADIFPTGWHGIEISGFQPGDSVAVFGAGPVGLMAAYSAQLRGASRVYVVDRVPERLRAAERIGATPIDFTAGDAVDQIIALNGDMVDRSVDAVGYQAVGKDNSTEQPNIVLENMIRVTRACGGLGIPGLYVPSDPGAGDASAAKGMISLSFGKLFEKGLSLGTGQCNVKAYNRQLRDLIIAGKARPSFVVSHEIGIDEAETAYEKFDKRVEGYTKVIIHPNGGFPSKRPPAGSSL

SEQ ID NO: 12 - protein, 194 aa, synthetic construct
MVDTSGVKIHPAVDNGIKPAQPGFAGGTLHCKCSTNPVRVAVRAQTAHNHVCGCTKCWKPEGAIFSQVAVVGRDALEVLEGAEKLEIVNAEAPIQRHRCRDCGVHMYGRIENRDHPFYGLDFVHTELSDEDGWSAPEFAAFVSSIIESGVDPSRMEAIRARLRELGLEPYDALSPPLMDAIATHIAKRSGALAA

SEQ ID NO: 13 - protein, 191 aa, synthetic construct
MANVSIHPAVDGGVVHGSTEGFAGGTLQCLCASNKVTVDVASQSAHNHACGCSKCWKPEGAKFSVVAVAPRDKVTVTAHPEKLKIVDESATIQRHACTGCGVHLYGRIENKDHAFYGLDFIHTELSQQSGWSPPGFAAFVSSIIETGTPPDQMDGVRARLTELGLTPYDCLSPALMDALSTNVARHKGLLH

SEQ ID NO: 14 - protein, 186 aa, synthetic construct
MSLPLHPSLNNGITKGSANFSGGKLRCKCSSSPVEVTLAGNVAHNHACGCSKCWKPEGAIFSVIGVIPKEQVSVTANADKLYIVDESAAIQRHACSGCGVHLYGRIEKEHPFKGLDFVHTELSSEKGWQEPQFAAFVSSIIEQGFDPSKMDAVRAQFKSIGLETYDALNPPLMDAIASWTAQKAKI

SEQ ID NO: 15 - protein, 191 aa, synthetic construct
MPVSLHPLVDNGITKGDANFPGGNLYCLCPQNKVTVAIKGNVAHNHACGCSKCWKPAGALFSVVGVVPKENLSVAANADKLEILDKAAAIQRYACKECGTHLFGRIEIDHPFKGLDFVHAELSDKKGWQEPQFAGFVSSIIEQGFHPNGMDEVRSKFQSLGLQTYDTLSPPLMDLIATYTGKKNGKLSANL

SEQ ID NO: 16 - protein, 369 aa, synthetic construct
MKSRAAVAFAPGKPLEIVEIDVAPPKKGEVLIKVTHTGVCHTDAFTLSGDDPEGVFPVVLGHEGAGVVVEVGEGVTSVKPGDHVIPLYTAECGECEFCRSGKTNLCVAVRETQGKGLMPDGTTRFSYNGQPLYHYMGCSTFSEYTVVAEVSLAKINPEANHEHVCLLGCGVTTGIGAVHNTAKVQPGDSVAVFGLGAIGLAVVQGARQAKAGRIIAIDTNPKKFDLARRFGATDCINPNDYDKPIKDVLLDINKWGIDHTFECIGNVNVMRAALESAHRGWGQSVIIGVAVAGQEISTRPFQLVTGRVWKGSAFGGVKGRSQLPGMVEDAMKGDIDLEPFVTHTMSLDEINDAFDLMHEGKSIRTVIRY

SEQ ID NO: 17 - protein, 378 aa, synthetic construct
MEIKQINSTIKSRAAVAFAPNQPLQIVEIDVEMPRKGEVLIRNTHTGVCHTDAFTLSGSDPEGVFPVVLGHEGAGVVVAVGEGVLSVKPGDHVIPLYTAECGECEFCRSGKTNLCVSVRDTQGKGLMPDCTTRFSYQGQPIYHYMGCSTFSEYSVVAEVSLAKINPEANHEQVCLLGCGVTTGIGAVHNTAKVQEGDSVAVFGLGAIGLAVVQGARQAKAGRIIAIDTNPAKFELAKQFGATDCLNPNDYDKPIKDVLLDINKWGIDHTFECIGNVNVMRQALESAHRGWGQSIIIGVAGAGQEISTRPFQLVTGRVWKGSAFGGVKGRSELPQMVEDSMKGDIQLEPFVTHTMPLDKINEAFELMHEGKSIRTVIHY

SEQ ID NO: 18 - protein, 386 aa, synthetic construct
MSAATVGKPIKCIAAVAYDAKKPLSVEEITVDAPKAHEVRIKIEYTAVCHTDAYTLSGSDPEGLFPCVLGHEGAGIVESVGDDVITVKPGDHVIALYTAECGKCKFCTSGKTNLCGAVRATQGKGVMPDGTTRFHNAKGEDIYHFMGCSTFSEYTVVADVSVVAIDPKAPLDAACLLGCGVTTGFGAALKTANVQKGDTVAVFGCGTVGLSVIQGAKLRGASKIIAIDINNKKKQYCSQFGATDFVNPKEDLAKDQTIVEKLIEMTDGGLDFTFDCTGNTKIMRDALEACHKGWGQSIIIGVAAAGEEISTRPFQLVTGRVWKGSAFGGIKGRSEMGGLIKDYQKGALKVEEFITHRRPFKEINQAFEDLHNGDCLRTVLKSDEIK

SEQ ID NO: 19 - protein, 379 aa, synthetic construct
MSTEGQIIKCKAAVAWEAGKDLSIEEIEVLPPRAHEVRVKVEFTGVCHTDAYTLSGADAEGSFPVVFGHEGAGVVESVGEGVESVKVGDSVVLLYTPECRECKFCLSGKTNLCGKIRATQGKGLLPDGTSRFRCKGKDLFHYMGCSSFSQYTVVADISVVKVQDEAPKDKTCLLGCGVTTGYGAAINTAKISKGDKIGVFGAGCIGLSVIQGAVSKGASEIIVIDINDSKKAWADQFGATKFVNPTTLPEGTNIVDYLIDITDGGFDYTFDCTGNVQVMRNALESCHKGWGESIIIGVAAAGKEISTRPFQLVTGRVWRGCAFGGIKGRTQMPSLVQDYLDGKIKVDEFITHRHDLDNINKAFHDMHAGNCIRAVITMH

SEQ ID NO: 20 - protein, 374 aa, synthetic construct
MANQVIRCKAAVAWEAGKPLSIEEIEVAPPKAHEVRIKILATAVCHTDAYTLSGADPEGCFPVILGHEGAGIVESVGEGVTKLKAGDTVIPLYIPQCGECKFCLNPKTNLCQKIRVTQGKGLMPDGTSRFTCKGKSVFHFMGTSTFSEYTVVADISVAKIDPSAPLDKVCLLGCGISTGYGAAVNTAKVEPGSTCAVFGLGGVGLAVIMGCKVAGASRIIGIDINKDKFAKAKEFGASECISPQDFSKSIQEVLVEMTDGGVDYSFECIGNVKVMRSALEAAHKGWGVSVVVGVAASGEEISTRPFQLVTGRTWKGTAFGGWKSVESVPKLVSEYMSKKIKVDEFVTGNLSFDQINQAFDLMHSGDSIRTVLKM

SEQ ID NO: 21 - protein, 375 aa, synthetic construct
ATVGKTIRCRAAVAWEAGKPLSMEEVEVAPPQAGEVRIKIVATGICHTDAYTLSGSDPEGVFPSVLGHEGAGIVESVGEGVTKFKSGDAVIPLYVPQCGECKFCKNPKTNLCQKIRLTQGKGLMPNGTSRFSCNGQVLFHFMGSSTFSEYTVVAEISLAKVHEKAPLDKVCLLGCAISTGYGAALNTAKVEAGSTCAVFGLGALGLAVIMGCQAAGASRIIAIDVNPDKFRIAKEFGATDLVNPKDHSKPVEQVLVEMTDGGVDYSFECVGNIAVMRAALEACHKGWGTSVIIGVAAAGQEISTRPFQLVTGRTWKGTAFGGYKSVESVPKLVEEYMNKKVKVDEFVTHTLPFEKIHEGFDLMGAGKSIRTVLNY

SEQ ID NO: 22 - protein, 278 aa, synthetic construct
MEMLEEHRCFEGWQQRWRHDSSTLNCPMTFSIFLPPPRDHTPPPVLYWLSGLTCNDENFTTKAGAQRVAAELGIVLVMPDTSPRGEKVANDDGYDLGQGAGFYLNATQPPWATHYRMYDYLRDELPALVQSQFNVSDRCAISGHSMGGHGALIMALKNPGKYTSVSAFAPIVNPCSVPWGIKAFSSYLGEDKNAWLEWDSCALMYASNAQDAIPTLIDQGDNDQFLADQLQPAVLAEAARQKAWPMTLRIQPGYDHSYYFIASFIEDHLRFHAQYLLK

SEQ ID NO: 23 - protein, 279 aa, synthetic construct
MTLAYETVSENRSFGGIQGVYRHQSQATGTPMTFAIYLPPDARHGKVPVLWYLSGLTCTHENAMTKAGAQEWAAEYGIAVIFPDTSPRGEGVANDETYDLGQGAGFYVDATEAPWAPHFRMWHYVTHELPELVFNNFPLDREAQGITGHSMGGHGALTIAMTFPERYRSVSAFAPIAHPSESDWGRKQFAAYLGDDKAAWKRHDSTILMREKGYPGEVLIDQGASDQFLDLLKPEALAHAMAERRQPGTFRMQQGYDHSYFFVQSFMADHIRWHAERLG

SEQ ID NO: 24 - protein, 299 aa, synthetic construct [sequence omitted]

SEQ ID NO: 25 - protein, 2380 aa, synthetic construct
MAVTVLPASSLTESVKQALRSTTTCSDATVLSLQTLLRGSPKMPEKPTKRTKSTREPAPAPSRTRTSRATKTKPANDTTLQSLADNDAAALSCQEKLVFATEVFNATLKTLTDAAKISTAKRQNNTPDAGNGPDAGIISAAECARLSLSTLRTLKNDPGNDQFPNMQLEQGLCVLAGKLISLGLNDVAYKELRLLKRRIQQHLDGGKAGKKTTEVKDAADEEGSKERMSDLLTFAHISNGKSLYGLLVPFHSNVMRLFAADRRASTIQKVCPSLQLSDSSSPAQVILAALKSGQLSNDKAALQLQLLSNTVLALCSGTSFSKDEASNSLKPTTSLALQLLSLEVRCLGWKLSGHVCDESKEVFDPLLRYFGSFSHRSKGIEKAEFASIYKTVTRLQTSIGEVKKKSSEAQIANQAAKLMTILGQLAFDAGCFDESMKLFTQAMNPLSKAQSLSLATVRCKIASVHFQASKVSRKFLDGALDSVSEATQSLGLQLRGSANDLDELLVEAARLKKLALAWFGEAITKGSDTESEKNEVASQIREYLQAFIRFLRRYVGRQPTEDGDEKEVEMFNKRISISRSIILAAIDSTVAVGKLSIMSQRPPWEEMLPILADCHRLLSTIESQDEKNAETSEPLGMALVKLSNLFWSRYIKEKEAGQGYRELIPLLKQSTLLLSSCSPSQRNTSFAALKFERMAHLYIEGNMYIESELMFRQSIEEYILSGTLDQIVKSSGGHNPTSVHQDPKSPGFMLGRVFSALLKMKLRRKGSHPSVVYDDVELEFEQRSLLIEWQMSLLLDMSSYSSNEEEFRLIFGSAVSSLLDLYPPDVYPIRHSRVILSALRLLLEQPTALDSSLIETLMDAGTKALDSGLQVRNDIDLASFAIHISNSLRIIIGFHRGKIDASELDDTLASWTSLVRQSHDWKTLLLCINDVDYWVLQLKALVDYTEIHGLWKAQLCTLELILRAAELQQSGDLSDPIIILSRLVLQNCRLGYCQKAGELLSRGEQYLAQSKVSSLATISYKVARVEYLLETGEPEKAATVLSAARSLYDKCQESELSNLTVLSKISWERLVADAAFVQSRLFSAQGSATQALYFAKLSVRLNCRIWAKVERLAQRKQDKMLPAAGSSDVEAVADGIAKLDLSQNGSSPDMSASYIQGAPFWPHLGSHHTCLLNLATLSAHHGLFQDAIYYGEQALKIDKTLDANARLLAAQTQLGCHWILSGHMSEGQDHLSAAAESSKQTQTSIETVSFQMGLASLYKTQGAYDKALRVLLEADKIITAVISADIPANLEAGGMVEIQEKMDKLRVRASSRRTPTPRTPTPTTTTTTRRTRATSSATTKTTKKAPAPKPTLPEVRSKSLLQLKGNILRQQADCLREFRDFERSAQTLAEARQFAVARESKITLEIGESEHLLADAIRRFASHAVYCVLPESTISLPSLKSPSKAADEPSLPPAKPSTRRTRAPAKTTRTKAQRASDDFSVMLSKASDCLASVFSDATILGSTLDSHAASRLMSRISMLSHATSPGIPATLAQSPANMNEIGRVGAFARERMAIDIDRQLADFADPLLWPTSFPSAVELDNDLCSNFTQDYVDILPETWNVLSLSLSADHTEFVVSRLQKDRSPFLLRLPLHRGNSEDDDEEQFTFEDGKEEMQELIKLANESAHAAKAQTDKLSKKEWWKTREALDRRMESVLQNIENIWFGGFRGVFSPLSRETTALARFASTFQSILDKHLPSRQKGGKAAGPRLTLHQNVVDLFIGLRDLEEQEEPEDTLMDLLYFVVDILQFQGERNAYDEIDFDMMVVDTLDALRGYHEAARDELAARPPRHTILVLDKALHLFPWESLPCLQGYPVCRVPSLECLRDRVLQFRKASSGAIVDRNSGAFVLNPTGDLRTTQTTFEQDLSRFKSWTAVVQREPTEDEFRDALEKKGLFLYFGHGSGAQYIRGRTVKRLTQCAVTFLMGCSSGTLTEAGEYEPYGTPMNYLHAGSPALVATLWDVTDRDIDRFTTTAFDAWGLVEKKDKKDKSRGQDVGLDTAIARSRVHQLQVLISNITTKWTFFPSCGTYLPPTIKTSTSPGFLAFYFLFSPKKYHILKMSVTTNATIASFGGKLLKLSHAATTTKCEMKFNLFLPPQAQTQKVPVLIYLSGLTCTAENCSEKGFFQHSASKKGIAVLYPDTSPRGLNIQGEDDAYDFGSGAGFYVDATKAPYNAGYNMYSYVTEELPQTVFAAFPQLDASRVSITGHSMGGHGALTLFLRNPGKYKSVSAFAPITNPTNCPWGQKAFKGYFGDDQQDKWKEHDATELIKKWSGGPLDILVDVGTGDNFYKQGQLLPENFEAAARDAGISGLNIRYQPDYDHSYYTMATFADDHVEHAAKYLFA

SEQ ID NO: 26 - protein, 282 aa, synthetic construct
MALKQISSNRCFGGLQKVFEHSSVELKCKMRFAVYLPPQAESGKCPALYWLSGLTCTEQNFISKSGYQQAASEHGLVVIAPDTSPRGCNIKGEDDSWDFGTGAGFYVNATEDPWKANYRMYSYVTEELPQLINANFPVDPQRMSIFGHSMGGHGALICALKNPGKYRSVSAFAPICNPVLCSWGKKAFSGYLGPDESKWKAYDATCLVKAYSGSQIDILIDQGKDDEFLSNGQLLPDNFIAACTEKKIPVVFRLQEGYDHSYYFIATFIADHIRHHAKYLNA

SEQ ID NO: 27 - protein, 282 aa, synthetic construct
MALKQLSSNKCFGGLQKVFEHDSVELKCKMKFAIYLPPKAETGKCPALYWLSGLTCTEQNFITKSGYHQAASEHGLVVIAPDTSPRGCNIKGEDESWDFGTGAGFYLDATEDPWKTNYRMYSYVTEELPQLINANFPVDPQRMSIFGHSMGGHGALICTLKNPGKYKSVSAFAPICNPVLCPWGKKAFSGYLGTDESKWKAYDATHLVKSYPGSQLDILIDQGKDDQFLSDGQLLPDNFIAACTEKKIPVVFRSQEGYDHSYYFIATFITDHIRHHAKYLNA

SEQ ID NO: 28 - protein, 288 aa, synthetic construct
MSKKLLFQFDTDATPSVFDVVVGYDGGADHITGYGNVTPDNVGAYVDGTIYTRGGKEKQSTAIFVGGGDMAAGERVFEAVKKRFFGPFRVSCMLDSNGSNTTAAAGVALVVKAAGGSVKGKKAVVLAGTGPVGMRSAALLAGEGAEVVLCGRKLDKAQAAADSVNKRFKVNVTAAETADDASRAEAVKGAHFVFTAGAIGLELLPQAAWQNESSIEIVADYNAQPPLGIGGIDATDKGKEYGGKRAFGALGIGGLKLKLHRACIAKLFESSEGVFDAEEIYKLAKEMA

SEQ ID NO: 29 - protein, 299 aa, synthetic construct
MEKVSILHLITAAKNASPFDVNMAFDAGFDKIVPYTNVELKEVTGLVQDAIFSRSPSGVKRESIFIGGRDIDVAMDMLETARKAMVPPFEVSVFADPSGAFTTAAAMMAKVEQHLIKNFGGDLSGRKVSVFGATGPVGGCTAVIAAKYGAEVELVAHRAVADVEEKAASYNQRYGIKIGYTDGSNDALKQQILQRTDIALCAAAAGIQVISLAQMAGSPTLKVVADVNAVPPTGAEGVDVFADGVAIPGTNAFGIGALAIGNVKYTTQHNLLKQMLEATEKKVYLDFLAAFETARNSIK

SEQ ID NO: 30 - protein, 286 aa, synthetic construct
MKKLLFQFDTDLHPSVFDTVVGYDGGADQVIAHGHLTPDNVGPLVEGTIFTRAPKDKKNTAIFVGGSDLVAGQNLLRAVRKKFFADFRVSVMLDSNGSNTTAAAGVAKLASSGTLAGKKAVVLAGTGPVGQRAAVMLAKEGCSEVVITSRQMARAEHACAEMKARFGVDLVPVEAFDDDARAAAIADAQIVFATGAAGVRLLEECHWRDRPDLELLADANATPPLGLGGTDMMDRGTDRHGKIVWGAIGFGTLKLAVHRACIAKLFERNDQVFDAEEIFALAKTMA

SEQ ID NO: 31 - protein, 399 aa, synthetic construct; identical to SEQ ID NO: 8

SEQ ID NO: 32 - protein, 412 aa, synthetic construct
MKALTYHGPHHVQVENVPDPGIEQADDIILRITATAICGSDLHLYRGKIPQVKHGDIFGHEFMGEVVETGKDVKNLQKGDRVVIPFVIACGDCFFCRMQQYAACENTNAGKGAALNKKQIPAPAALFGYSHLYGGVPGGQAEYVRVPKGNVGPFKVPPLLSDDKALFLSDILPTAWQAAKNAQIQQGSSVAVYGAGPVGLLTIACARLLGAEQIFVVDHHPYRLRFAADRYGAIPINFDEDSDPAQSIIEQTAGHRGVDAVIDAVGFEAKGSTTETVLTNLKLEGSSGKALRQCIAAVRRGGIVSVPGVYAGFIHGFLFGDAFDKGLTFKMGQTHVHAWLGELLPLIEKGLLKPEEIVTHYMPFEEAARGYEIFEKREEECRKVILVPGAQSAEAAQKAVSGLVNAMPGGTI

SEQ ID NO: 33 - protein, 393 aa, synthetic construct
MKAVTWHGRRDVRVDTVQDPRIQEPTDAIIEVTSTNICGSDLHLYEVLGAFMNAGDILGHEAMGVVREVGAGVSNLAVGDRIVVPFQISCGHCFMCDEQLYTQCETTQVREQGMGAALFGYSELYGEVPGGQAEYLRIPQAQFTHIKVPEGPPDSRFVYLSDVLPTAWQGVAYAGIPDGGSVTVLGLGPIGDMAARIATHLGYRVIAVDRVPERLARATARGIETIDMTGLSGSVGDAVRDLTDGRGTDSVIDAVGMEAHGSPVAQAAQTAAAFLPDFVAKPFMQKAGVDRLGALYSAIDCVRRGGTISLSGVYGGMADPMPMLTLFDKQIQLRMGQANVKKWVDDIMPLLTDADPLGVDSFATHVLPLDQAPHAYDIFQKKQDGAVKVILQP

SEQ ID NO: 34 - protein, 949 aa, synthetic construct
MDKQADYGTPASRTTEQQVTLEIDGMQVTVAKGTSIMRAAMEAGVSIPKLCATDTLEPFGSCRLCLVEIEGRRGYPASCTTPVDEGLKVHTQTPKLADIRRGVMELYISDHPLDCLTCSANGDCELQDMAGAVGLREVRYGYDGSNHLHAEKDLSNPYFQFDPSKCIVCSRCVRACEETQGTFALTIQGRGFDSKVAAGNFDNFLESECVSCGACVTACPTATLMEKTVIEHGQPEHSVITTCAYCGVGCSFRAEMKGEQVVRMVPDKNGGANHGHSCVKGRFAWGYATHRDRITTPMIRKSIHDPWQEVSWEEAITYAASELKRIQAKHGRNSIGAITSSRCTNEETYLVQKLVRAAFGNNNVDTCARVCHSPTGYGLKQTLGESAGTQTFDSIMKSDVIMVIGANPTDGHPVFGSQMKRRLREGAKLIIADPRAIDLVSGPHVKADYHLKLRPGTNVALITALAHVVVTEGLVDEAFVRERCEWDSYQYWSEFVAQPEHSPEAMQDVIGVPAQDLRAAARLYATGGNAAIYYGLGVTEHSQGSTMVMGIANLAMATGNIGREGVGVNPLRGQNNVQGACDMGSFPHEFPGYRHVSDDTTRALFEAAWGRPLDKEPGLRIPNMLDFAIHGSFKALYCEGEDIAQSDPNTQHVTQALSSMECVIVQDLFLNETAMYAHVFLPGCSFLEKNGTFTNAERRISPVRRVMTPKNGYEDWQITAMLSEALGYPMPYRHASEILDEIARLTPTFHGVSFKKLEEMGSIQWPCNEEHPNGTPIMHVDEFVRGKGRFMITEYVPTSERVNEKYPLILTTGRILSQYNVGAQTRRTDNVTWHPEDMVEIHPHDAEDRGIKDGDWVGITSRAGNTVLRAKITERVQPGVIYTTFHHPESGANVITTDNSDWATNCPEFKVTAVQVTRVSQLSDWQRRYQEFSNSQIALVKQRDMARMG

SEQ ID NO: 35 - protein, 1016 aa, synthetic construct
MQVSRRQFFKICAGGMAGTTAAALGFAPSVALAETRQYKLLRTRETRNTCTYCSVGCGLLMYSLGDGAKNAKASIFHIEGDPDHPVNRGALCPKGAGLVDFIHSESRLKFPEYRAPGSDKWQQISWEEAFDRIAKLMKEDRDANYIAQNAEGVTVNRWLSTGMLCASASSNETGYLTQKFSRALGMLAVDNQARVUHGPTVASLAPTFGRGAMTNHWVDIKNANLVVVMGGNAAEAHPVGFRWAMEAKIHNGAKLIVIDPRFTRTAAVADYYAPIRSGTDIAFLSGVLLYLLNNEKFNREYTEAYTNASLIVREDYGFEDGLFTGYDAEKRKYDKSSWTYELDENGFAKRDTTLQHPRCVWNLLKQHVSRYTPDVVENICGTPKDAFLKVCEYIAETSAHDKTASFLYALGWTQHSVGAQNIRTMAMIQLLLGNMGMAGGGVNALRGHSNIQGLTDLGLLSQSLPGYMTLPSEKQTDLQTYLTANTPKPLLEGQVNYWGNYPKFFVSMMKAFFGDKATAENSWGFDWLPKWDKGYDVLQYFEMMKEGKVNGYICQGFNPVASFPNKNKVIGCLSKLKFLVTIDPLNTETSNFWQNHGELNEVDSSKIQTEVFRLPSTCFAEENGSIVNSGRWLQWHWKGADAPGIALTDGEILSGIFLRLRKMYAEQGGANPDQVLNMTWNYAIPHEPSSEEVAMESNGKALADITDPATGAVIVKKGQQLSSFAQLRDDGTTSCGCWIFAGSWTPEGNQMARRDNADPSGLGNTLGWAWAWPLNRRILYNRASADPQGNPWDPKRQLLKWDGTKWTGWDIPDYSAAPPGSGVGPFIMQQEGMGRLFALDKMAEGPFPEHYEPFETPLGTNPLHPNVISNPAARIFKDDAEALGKADKFPYVGTTYRLTEHFHYWTKHALLNAILQPEQFVEIGESLANKLGIAQGDTVKVSSNRGYIKAKAVVTKRIRTLKANGKDIDTIGIPIHWGYEGVAKKGFIANTLTPFVGDANTQTPEFKSFLVNVEKV

SEQ ID NO: 36 - protein, 376 aa, synthetic construct
MSKGKVLLVLYEGGKHAEEQEKLLGCIENELGIRNFIEEQGYELVTTIDKDPEPTSTVDRELKDAEIVITTPFFPAYISRNRIAEAPNLKLCVTAGVGSDHVDLEAANERKITVTEVTGSNVVSVAEHVMATILVLIRNYNGGHQQAINGEWDIAGVAKNEYDLEDKIISTVGAGRIGYRVLERLVAFNPKKLLYYDYQELPAEAINRLNEASKLFNGRGDIVQRVEKLEDMVAQSDVVTINCPLHKDSRGLFNKKLISHMKDGAYLVNTARGAICVAEDVAEAVKSGKLAGYGGDVWDKQPAPKDHPWRTMDNKDHVGNAMTVHISGTSLDAQKRYAQGVKNILNSYFSKKFDYRPQDIIVQNGSYATRAYGQKK

SEQ ID NO: 37 - protein, 894 aa, synthetic construct
MIKVIVNGIGYEVPEDITVLQACQKVGIDIPTLCHDERLEPHASCRLCVVEVEGMRNLPTSCSLKVYDGMVIQTDSQKVVSARKDVLDLLFSNHPNDCLTCKKSGECKLQDYCYEYGILEGGYKGEKRSLPIDDSNHFYFYDPNKCILCGKCVRVCNELQCTNAITIDERGFDSLVSTPFRKGLENSTCVSCGNCVSVCPVGALTPKTRENFRHWDTKRTKTTCSYCGVGCQFELISTNGKIVGVQPVNGKPNDGLLCVKGKFGYPFINHPDRLKNPLIRKNGVLEEASWNEAISLIASKIKETKENYGADAFGGFSSARCTNEENYLFQKLFRAVIGTNNVDHCARLUHASTVAGLATTLGSGAMTNSVRETVDNDVLFVIGSNTTENHPVIGTQMKQAKKKGAKIIVADPRRIELADQADVFLQIKPGTNIALLNGMMNYIIENELYDKDYIDKRTENFEEVKQVVKDYTPEKVAEICEVNKDDIIKAARIYAESDRAGIYYAMGITQHTTGTHNVIAISNLALMCGNIGKENAGVNPLRGQNNVQGACDMGCLPSDLPGYQKVFKEEIAEKFEKAWGVSLSRQVGLAISEMIHGAETGDIRFLYIMGENPMVSDPDITHVQHALESVDFLVVQDIFLTETAEFADVVLPAASFAEKDGTFSNTERRVQRVRKAIEPVGNAKADWQILMEIMNKAGYNKIYLDTSEIMDEIASVTPSYGGITYERIEDEGIQWPCPTKEHPGTKYLHKEAIARGRGLFFPVEYTGSAETKSEEYPFILTTGRVLYHYHTRTMTGRVDGLNKKVPSSFIELNEVTANKMGIKDGEVVKVTSRRGNINIAVKVTDIVDEDVVFIPFHFAEGAANYLTNTELDPIAKIPELKVAAVKIEKLKESC

SEQ ID NO: 38 - protein, 1032 aa, synthetic construct
MGDIMRPIPFEELLTRIFDEYQQQRSIFGIPEQQFYSPVKGKTVSVFGETCATPVGPAAGPHTQLAQNIVTSWLTGGRFIELKTVQILDRLELEKPCIDAEDECFNTEWSTEFTLLKAWDEYLKAWFALHLLEAMFQPSDSGKSFIFNMSVGYNLEGIKQPPMQQFIDNMMDASDHPKFAQYRDTLNKLLQDDAFLARHGLQEKRESLQALPARIPTSMVHGVTLSTMHGCPPHEIEAICRYMLEEKGLNTFVKLNPTLLGYARVREILDVCGFGYIGLKEESFDHDLKLTQALEMLERLMALAKEKSLGFGVKLTNTLGTINNKGALPGEEMYMSGRALFPLSINVAAVLSRAFDGKLPISYSGGASQLTIRDIFDTGIRPITMATDLLKPGGYLRLSACMRELEGSDAWGLDHVDVERLNRLAADALTMEYTQKHWKPEERIEVAEDLPLTDCYVAPCVTACAIKQDIPEYIRLLGEHRYADALELIYQRNALPAITGHICDHQCQYNCTRLDYDSALNIRELKKVALEKGWDEYKQRWHKPAGSGSRHPVAVIGAGPAGLAAGYFLARAGHPVTLFEREANAGGVVKNIIPQFRIPAELIQHDIDFVAAHGVKFEYGCSPDLTVEQLKNQGFHYVLIATGTDKNSGVKLAGDNQNVWKSLPFLREYNKGTALKLGKHVVVVGAGNTAMDCARAALRVPGVEKATIVYRRSLQEMPAWREEYEEALHDGVEFRFLNNPECFDADGTLTLRVMSLGEPDEKGRRRPVETNETVTLHVDSLITAIGEQQDTEALNAMGVPLDKNGWPDVDHNGETRLTDVFMIGDVQRGPSSIVAAVGTARRATDAILSRENIRSHQNNKYWNNVNPAEIYQRKGDISITQVNSDDRDAFVAQEAARCLECNYVCSKCVDVCPNRANVSIAVPGFQNRFQTLHLDAYCNECGNCAQFCPWNGKPYKDKITVFSLSQDFDNSSNPGFLVEDCRVRVRLNNQSWVLNIDSEGQFDNVPPELNDMCRIISHVHQHHHYLLGRVEV

SEQ ID NO: 39 - protein, 575 aa, synthetic construct
MAIDAKDPVRDHGAASRPIAGRGVEGPSKMSKHGDMTSVIDLTREKGTGPTRTRRPLYVDLLPPCRAACPAGEDIQGWLALAQAGNYRKAWELLVRENPFPAVHGRVCYHPCESHCNRGDYDAPVSIHAIERFLGDLASAGGWPFPPAAEPSGKRVLVVGAGPCGLSASYHLARLGHAVEVHEAGPLAGGMMHFGIPAYRLPREALAKEVERIERMGVRFVFDHKVEELLAEKAAGGFDAVLVAIGAQIGKHVDIPARDAARVLDAVSLLHQVGGEERPLLGRRVVIYGGGNVAMDAARTAKRLGAEEALIVYRRDRAHMPARAFEADEALSEGIRIRWLTTIKEIVGEELTVERMELGSDGRPRPTGQYDTLRADAVVLAIGQETDSRFLRRVPGIVFGKDGAVIVDQNRMTGHPGIFAGGDAVPGDQTVTDAVGQGKKAARSIDAWLRGSVYAEPAPPSGVSFPMLHLPVYRDVAPGHQPERPPAERTSGFAEVVAGLSETEARREAERCFSCGICFECDNCYAACPEDAILKLGPGKRYRFLYDRCTGCAVCFDQCPCHAIEMIPEPLGAES

SEQ ID NO: 40 - protein, 619 aa, synthetic construct
MSTMDTWRGSKASETHKAFMGWGGLTVNDDTVDILDMLRAYYDVAAGESCGQCFPCRSGLKRIAARLAEICQGQERPDDQNYLRELAAMVRTSARCDIGQTSPQPLLDVLEQAPHLLKARKTTGGNYTSLITAPCVNACPGHVNIPDYIEEIRFRRFEKGLELVMNNCPMPGTIGRVCERPCESACKRGLKGAPVAIRNLKRFLFDRNAALNNPPEPQSLPATAKKVAIIGGGPAGLSCAYYLSLLGAAPTIFERHDVCGGMAKFGIPDFRLPPAVLVREVNVVAAAGCEIRNGVEIGRDISLDQLHEEGFEAVFIAAGAPHAPGMRCEGEDSCPQGYLSGIHYLHEATRGRQAVTGTRLVVVGGGNVAMDCARTALRHGFKEVRVVYRRTEAEMPADPVEIEEAKEEGTLFTFLAAPLRIESKDGRVTGLVCQKMELGAADDSGRRRPVAVEGADYELPCDAIVYAIGQKVALEVILKGKDGALNKYRTLDAHEITGEVTTLPRIFGGGDCVTGPSSLIAALAAGKRAATHIAAHLNDSAEGPSSREELEQMLMGVNMLDAEEVAPLEDPTPAMPIHAIPLRERLSGFTEVETDPLEWEAVRESSRCLRCLRVVMTAH

SEQ ID NO: 41 - protein, 209 aa, synthetic construct
MALTQMALDSLDFDATVALAEKVAPHVDILEIGTPCIKHNGIKLLETLRAKFPNNKILVDLKTMDAGFYEAEPFYKAGADITTVLGVADLGTIKGVIDAANKYGKKAQIDLINVGDKAARTKEVAKLGAHIIGVHTGLDQQAAGQTPFADLATVTGLNLGLEVSVAGGVKPATVAQVKDAGATIIVAGAAIYGAADPAAAAAEITGLAK

SEQ ID NO: 42 - protein, 210 aa, synthetic construct
MELQLALDLVNIPEAIELVKEVEQYIDVVEIGTPVVINEGLRAVKEIKEAFPQLKVLADLKIMDAGGYEIMKASEAGADIITVLGATDDATIKGAVEEAKKQKKKILVDMINVKDIESRAKEIDALGVDYICVHTGYDLQAEGKNSFEELTTIKNTVKNAKTAIAGGIKLDTLPEVIQQKPDLVIVGGGITSAADKAETASKMKQLIVQG

SEQ ID NO: 43 - protein, 228 aa, synthetic construct
MAKPLVQMALDSLDFDQTVALATTVAPHVDILEIGTPCIKYNGIKLLETLRAKFPNNKILVDLKTMDAGFYEAEPFYKAGADIVTVLGTADIGTIKGVIDVANKYGKKAQVDLINVTDKAARTKEVAKLGAHIIGVHTGLDQQAAGQTPFADLNLVSSLNLGVDISVAGGVKATTAKQVVDAGATIVVAGAAIYGAADPAAAAAEISAAAKGTQSSGGLFGWLKKLFS

SEQ ID NO: 44 - protein, 181 aa, synthetic construct
MNKYQELVVNKLTNVINNTAEGYDDKILSMVDAAGRTFLGGAGRSLLVSRFFAMRLVHAGYQVSMVGEVVTPSIQAGDLFIVISGSGSTETLMPLVRKAKSQGAKVIVISMKAQSPMAELADLVVPIGGNDAHAFDKTHGMPMGTIFELSTLWFLEATIAKLIDQKGLTEEGMRAIHANLE

SEQ ID NO: 45 - protein, 185 aa, synthetic construct
MKTTEYVAEILNELHNSAAYISNEEADQLADHILSSHQIFTAGAGRSGLMAKSFAMRLMHMGFNAHIVGEILTPPLAEGDLVIIGSGSGETKSLIHTAAKAKSLHGIVAALTINPESSIGKQADLIIRMPGSPKDQSNGSYKTIQPMGSLFEQTLLLFYDAVILKLMEKKGLDSETMFTHHANLE

SEQ ID NO: 46 - protein, 181 aa, synthetic construct
MNKYQELVVSKLTNVINNTAEGYDDKILSLVDAAGRTFIGGAGRSLLVSRFFAMRLVHAGYQVSMVGEVVTPSIQAGDLFIVISGSGSTETLMPLVKKAKSQGAKIIVISMKAQSPMAELADLVVPVGGNDANAFDKTHGMPMGTIFELSTLWFLEATIAKLVDQKGLTEEGMRAIHANLE

SEQ ID NO: 47 - protein, 549 aa, synthetic construct
MKNINPTQTAAWQALQKHFDEMKDVTIADLFAKDGDRFSKFSATFDDQMLVDYSKNRITEETLAKLQDLAKECDLAGAIKSMFSGEKINRTENRAVLHVALRNRSNTPILVDGKDVMPEVNAVLEKMKTFSEAIISGEWKGYTGKAITDVVNIGIGGSDLGPYMVTEALRPYKNHLNMHFVSNVDGTHIAEVLKKVNPETTLFLVASKTFTTQETMTNAHSARDWFLKAAGDEKHVAKHFAALSTNAKAVGEFGIDTANMFEFWDWVGGRYSLWSAIGLSIVLSIGFDNFVELLSGAHAMDKHFSTTPAEKNLPVLLALIGIWYNNFFGAETEAILPYDQYMHRFAAYFQQGNMESNGKYVDRNGNVVDYQTGPIIWGEPGTNGQHAFYQLIHQGTKMVPCDFIAPAITHNPLSDHHQKLLSNFFAQTEALAFGKSREVVEQEYRDQGKDPATLDYVVPFKVFEGNRPTNSILLREITPFSLGALIALYEHKIFTQGVILNIFTFDQWGVELGKQLANRILPELKDDKEISSHDSSTNGLINRYKAWRG

SEQ ID NO: 48 - protein, 555 aa, synthetic construct
MTNPTNCPIWHDLSAHYQEVLPLQMRDMFTKDGRRFEKFSLEAEGLLLDYSKHRITDETLPLLFKLARDSKVEEWRDRMFAGEKINFTENRAVLHTALRNRSNTPVYVDGKDVMPDVNRVLAQMRKFSTSIRSGEWKGYSGKRITDVVNIGIGGSDLGPVMVCGALKPYAQAGLNAHFVSNIDGTHLAQTLERCDPETTLFIVASKTFTTQETMTNARSARSWFLQAAKDEAHVAKHFVAISTNADEVGKFGIDAANMFEFWDWVGGRYSLWSAIGLSIAIYIGMDHFEELLQGGYEIDRHFKNAPLEQNIPVIMALLGIWYNNFFGADSLAILPYDQGLARFPAYLQQADMESNGKFVARDGRIVQCTTGPIIWGEAGTNGQHAFYQLIHQGNRLIPCDFMMPLQSHYSMGKNGNEHHLILLANCFAQTSALMQGKTLDEAKAELVAQGLTGEALETLLPHKVFEGNRPSTTILFDKLTPKTLGKLIAIYEHKIFVQGIIWNINSFDQWGVEYGKQIAKKILPQLSEDQASTEYDSSTNGLMNYFKSRTQSSGT

SEQ ID NO: 49 - protein, 554 aa, synthetic construct
MSNNSFTNFKLATELPAWSKLQKIYESQGKTLSVKQEFQKDAKRFEKLNKTFTNYDGSKILFDYSKNLVNDEIIAALIELAKEANVTGLRDAMFKGEHINSTEDRAVYHVALRNRANKPMYVDGVNVAPEVDSVLKHMKEFSEQVRSGEWKGYTGKKITDVVNIGIGGSDLGPVMVTEALKHYAGVLDVHFVSNIDGTHIAETLKVVDPETTLFLIASKTFTTAETITNANTAKNWFLSKTGNDPSHIAKHFAALSTNETEVAKFGIDTKNMFGFESWVGGRYSVWSAIGLSVALYIGYDNFEAFLKGAEAVDNHFTQTPLEDNIPLLGGLLSVWYNNFFGAQTHLVAPFDQYLHRFPAYLQQLSMESNGKSVTRGNVFTDYSTGSILFGEPATNAQHSFFQLVHQGTKLIPSDFILAAQSHNPIENKLHQKMLASNFFAQAEALMVGKDEEQVKAEGATGGLVPHKVFSGNRPTTSILAQKITPATLGALIAYYEHVTFTEGAIWNINSFDQWGVELGKVLAKVIGKELDNSSTISTHDASTNGLINQFKEWM

SEQ ID NO: 50 - protein, 558 aa, synthetic construct
MAALTRNPQFQKLLEWHRANSANLKLRELFEADPERFNNFSLNLNTNHGHILVDYSKNLVNKEVMQMLVELAKSRGVEAARDNMFSGSKINYTENRAVLHVALRNRSNTPIKVDGKDVMPEVNRVLDKMKSFCQRVRSGDWKGYTGKSITDIINIGIGGSDLGPLMVTEALKPYSKGGPRVWFVSNIDGTHIAKTLASLSPETSLFIIASKTFTTQETITNAETAKEWFLEAAKDPSAVAKHFVALSTNTAKVKEFGIDPQNMFEFWDWVGGRYSLWSAIGLSIALHVGFDHFEQLLSGAHWMDQHFLKTPLEKNAPVLLALLGIWYINCYGCETHALLPYDQYMHRFAAYFQQGDMESNGKYITKSGARVDHQTGPIVWGEPGTNGQHAFYQLIHQGTKMIPCDFLIPVQTQHPIRKGLHHKILLANFLAQTEALMKGKLPEEARKELQAAGKSPEDLEKLLPHKVFEGNRPTNSIVFTKLTPFILGALIAMYEHKIFVQGIMWDINSFDQWGVELGKQLAKKIEPELEGSSAVTSHDSSTNGLISFIKQQRDTKLE

SEQ ID NO: 51 - protein, 325 aa, synthetic construct
MSARDTVLVTGASGFLGRAVVRDLQDAGYAVRTFQRRPSGVAGAEDVLGSVTDAGAVRGAVDGADAVVHLAAKVSLTGDPADFERINVAGTADLLDAARAAGASRFVHVSSPSVAHAGTSIVGDDAEPADPAHARGEYARTKALGERLALAADSGAMPLVVVRPHLVWGPGDTQLVERVVERARAGRLPLLGAGQALIDTTYVDNAASAIVAALERAPEVHGNAYVVTNGEPRAVAELLTGICEAAGVRPPAWSVPPAVARAAGGLVERVWAVRPGADEPPMTRFLAEQLSTAHWFDQRRTRADLRWTPSVTLDEGFARLAASYR

SEQ ID NO: 52 - protein, 486 aa, synthetic construct
MVSEIKTLVTFFGGTGDLAKRKLYPSVFNLYKKGYLQKHFAIVGTARQALNDDEFKQLVRDSIKDFTDDQAQAEAFIEHFSYRAHDVTDAASYAVLKEAIEEAADKFDIDGNRIFYMSVAPRFFGTIAKYLKSEGLLADTGYNRLMIEKPFGTSYDTAAELQNDLENAFDDNQLFRIDHYLGKEMVQNIAALRFGNPIFDAAWNKDYIKNVQVTLSEVLGVEERAGYYDTAGALLDMIQNHTMQIVGWLAMEKPESFTDKDIRAAKNAAFNALKIYDEAEVNKYFVRAQYGAGDSADFKPYLEELDVPADSKNNTFIAGELQFDLPRWEGVPFYVRSGKRLAAKQTRVDIVFKAGTFNFGSEQEAQEAVLSIIIDPKGAIELKLNAKSVEDAFNTRTIDLGWTVSDEDKKNTPEPYERMIHDTMNGDGSNFADWNGVSIAWKFVDAISAVYTADKAPLETYKSGSMGPEASDKLLAANGDAWVFKG

SEQ ID NO: 53 - protein, 489 aa, synthetic construct
MPDVRVLPCTLALFGALGDLALRKLFPALYQLDRENLLHRDTRVLALARDEGAPAEHLATLEQRLRLAVPAKEWDDVVWQRFRERLDYLSMDFLDPQAYVGLREAVDDELPLVAYFATPASVFGGICENLAAAGLAERTRVVLEKPIGHDLESSREVNEAVARFFPESRIYRIDHYLGKETVQNLIALRFANSLFETQWNQNHISHVEITVAEKVGIEGRWGYFDQAGQLRDMVQNHLLQLLCLIAMDPPSDLSADSIRDEKVKVLRALEPIPAEQLASRVVRGQYTAGFSDGKAVPGYLEEEHANRDSDAETFVALRVDIRNWRWSGVPFYLRTGKRMPQKLSQIVIHFKEPPHYIFAPEQRSLISNRLIIRLQPDEGISLQVMTKDQGLGKGMQLRTGPLQLSFSETYHAARIPDAYERLLLEVTQGNQYLFVRKDEVEFAWKWCDQLIAGWERLSEAPKPYPAGSWGPVASVALVARDGRSWYGDF

SEQ ID NO: 54 - protein, 789 aa, synthetic construct
MLLAAMCLALLGCLQAQELKGHVSIILLGATGDLAKKYLWQGLFQLYLDEAGKGHSFSFHGAALTAPQQGQKLMDKVLESLSCPKDLVPSRCDELKGQFLQLSQYRQLKTVEDYQTLNKDIETQVQQDGLWEAGRIFYFSVPPFAYADIARNINSSCRPHPGAWLRVVFEKPFGHDHLSAQQLASELGSFFQEEEMYRVDHYLGKQAVAQILPFRDQNRKALDGLWNRHHVERVEIILKETIDAEGRASFYEEYGVIRDTLQNHLTEILTLVAMELPLNISSSAAVLQHKLWAFQALRGLQKSSAILGQYQAYSGQVRRELQKPDGFQSLTPTFAGVLVHIDNLRWEGVPFILMSGKALDERVGYVRIVFKNRAYCTQSERHWVPEQSRCLPQQIIFYIGHGELGHPAILVSRNLFKPSLPTQKWKEVQDQPGLRLFGRPLSDYYAYRPVREQDAYSTLLSHIFHCRKESFITTENLLASWVFWTPLLDSLAFEVPRPYPGGAENGQLLDFEFSGGQLTFSQQQLEVLIPDLGSVPKPSDFQVLGARYRQSPLITAWPEELISKLASDIEAAAVQAVRHFGKFHLALSGGSSPIALFQQLATGHYSFPWAHTHLWLVDERCVPLSDPDSNFQGLQAHLLQHVRVPYYNIHPMPVHLHQRLCAEEDQGAQTYASEISALVANSSFDLVLLGMGTDGHTASLFPQSPTGLDGDQLVVLTESPFRPHQRMSLSLPLINRAKKVAVLVMGRTKREITTLVSRVGHEPKKWPISGVVPLSGQLVWYMDYEAFLG

SEQ ID NO: 55 - protein, 797 aa, synthetic construct
MKCPGVWGMLTVTMCVVFLGCPQAQELQGHVSVILLGATGDLAKKYLWQGLFQLFLDEAGKGHSFSFHGAALTAPKQGQELMAKALESLSCPRDMAPSRCAELQAQFLRLSRYRQLKTAEDYQALGRDIEAQVQQEGLREAGRMFYFSVPPFAYADIARNINSSCRPGPGAWLRVVLEKPFGHDHLSAQQLATELGSFFQEEEMYRVDHYLGKQAVAQILPFRDQNRRALDSLWNRHHVERVEIIMKETVDAEGRTSFYEEYGVIRDTLQNHLTEILTLVAMELPANVSCSEAVLRHKLQAFRALRRLQRGSAVVGQYQTYSEQVRRELRKPAGSPSLTPTFAGVLVHVDNLRWEGVPFILMSGKALDERVGYVRVLFKNQAFCAQSEKHWAPAQSRCLPRQIIFYIGHGELGHPAVLVSRNLFRPFLPAQSWREVEDRPGLQLFGRPLSDFYAFSPVKERDAYSILLSHIFHARKESFVPTEHLLASWVFWTPLLESLAREVPRLYPGGADSGRLLDFEFSGSHLSFSLGQPEQLVPGPGSTPRPSDFQVLGAKYRESPLISAWPDELISKLASDIEAAAVQAVRRVGTFHLALSGGSSPIALFQQLASGHYGFPWAHTHLWLVDERCVPLSDPESNFQGLQAHLLQHVRVPYYNIHPMPVNLHQRLCAEEDRGAQAYASEISALVTNCSFDLVLLGMGTDGHTASLFPQSPTGLDGEQLVVLTESPSRPHQRMSLSLPLINRAKKVAVLVMGRTKRDITLLVSRVGREPKKWPISGVLPTSGQLVWYMDYEAFLG

SEQ ID NO: 56 - protein, 491 aa, synthetic construct
MAVTQTAQACDLVIFGAKGDLARRKLLPSLYQLEKAGQLNPDTRIIGVGRADWDKAAYTKVVREALETFMKETIDEGLWDTLSARLDFCNLDVNDTAAFSRLGAMLDQKNRITINYFAMPPSTFGAICKGLGEAKLNAKPARVVMEKPLGTSLATSQEINDQVGEYFEECQVYRIDHYLGKETVLNLLALRFANSLFVNNWDNRTIDHVEITVAEEVGIEGRWGYFDKAGQMRDMIQNHLLQILCMIAMSPPSDLSADSIRDEKVKVLKSLRRIDRSNVREKTVRGQYTAGFAQGKKVPGYLEEEGANKSSNTETFVAIRVDIDNWRWAGVPFYLRTGKRLPTKCSEVVVYFKTPELNLFKESWQDLPQNKLTIRLQPDEGVDIQVLNKVPGLDHKHNLQITKLDLSYSETFNQTHLADAYERLLLETMRGIQALFVRRDEVEEAWKWVDSITEAWAMDNDAPKPYQAGTWGPVASVAMITRDGRSWNEFE

SEQ ID NO: 57 - protein, 493 aa, synthetic construct
MKVIDPCTLVLFGASGNLSRIKLMPGLFRLDQAGRLPENMAILSVGRGQVSREDWLADIKSMLDAKFPKGYDQAVFKRFIERHHYHANPPDDATSFTRMKETLSNEAIFPQNLAFFLSVRPSDFATIVDQLAGVGLTKEDKYWRRVVVEKPFGTDLKSAQELQSSITKHLKESQVYRIDHYLGKSALQNIMLQRFANTILEPLWNNQYIDHVQITNTEQLGVGERTQFYDATGALRDMIQSHVLQTLALTAMEQPASLSPDDVRAEKIKVLEAIRPIPVDQLEKNAFRAQYSAGEVKGEQVPGYLEELGDSSSVVETYAALKLFIDNPRWQGVPFYIRTAKRLHEADTRIAIRFKKAPLQLGKGQEQNWLIIGIQPRECIKLEIQSKIPGLDVATRSIELDGANRQEGDETIDAYEALLLNLMEGDNSHYLHISEVEAQWRLVDPVIEAWSKDRNPVHQYPAGSSDPEASRVIFEHEDQFWRYSIQLGGDKQA

SEQ ID NO: 58 - protein, 505 aa, synthetic construct
MSEGPVKFEKNTVISVFGASGDLAKKKTFPALFGLFREGYLDPSTKIFGYARSKLSMEEDLKSRVLPHLKKPHGEADDSKVEQFFKMVSYISGNYDTDEGFDELRTQIEKFEKSANVDVPHRLFYLALPPSVFLTVAKQIKSRVYAENGITRVIVEKPFGHDLASARELQKNLGPLFKEEELYRIDHYLGKELVKNLLVLRFGNQFLNASWNRDNIQSVQISFKERFGTEGRGGYFDSIGIIRDVMQNHLLQIMTLLTMERPVSFDPESIRDEKVKVLKAVAPIDTDDVLLGQYGKSEDGSKPAYVDDDTVDKDSKCVTFAAMTFNIENERWEGVPIMMRAGKALNESKVEIRLQYKAVASGVFKDIPNNELVIRVQPDAAVYLKFNAKTPGLSNATQVTDLNLTYASRYQDFWIPEAYEVLIRDALLGDHSNFVRDDELDISWGIFTPLLKHIERPDGPTPEIYPYGSRGPKGLKEYMQKHKYVMPEKHPYAWPVTKPEDTKDN

SEQ ID NO: 59 - protein, 475 aa, synthetic construct
MLSIIVFGASGDLATKMTFPALFALYVRKIIPEDFQIIGYARSKLSQEAANKIVTAHIPIDDTVGASQKALNTFVEHYKYVPGTYDKPESFEMLNSIIAEKETAPASECTRIFYLVLPPHLFAPVSELIKSKAHPNGMVTRLIVEKPIGFDYKSADAILSDLSKHWSAKDTFKVDHFLGEDMIDGFTAIRFANSMFEPIWNREHIESVRVDFREDFGCEGRGGYFEGAGILRDVVQNHLLQLLTLLCIEEPKSQDAEDIIKCKVDFLKSLHPVSKEDIVYGQYTKSANGKVPGYRELDGVADDSEVSTFCALQLRSEAPRWKGIPIIISAGKGLDRDYFEARITFKRREGGMFPTVDSSNVLVLRVYPKEFIALKGHIKQPGFSRQIVPVTLDVKYPEAFPDTWIHKAYEVVIADAINGKHTHFISDDEVRTSWKIFDDVLDTTGDLSPLPYAFGSHHGPDATLEFFKKRNLEWD

SEQ ID NO: 60 - protein, 515 aa, synthetic construct
MAEQVALSRTQVCGILREELYQGDAFHQADTHIFIIMGASGDLAKKKIYPTIWWLFRDGLLPEDTFIVGYARSRLTVDDIRKQSEPFFKATPEERPKLEEFFARNSYVAGQYDDAASYKHLNSHMNALHQGMQANRLFYLALPPTVYEAVTKNIQETCMSQTGWNRIIVEKPFGRDLQSSNQLSNHISSLFREDQIYRIDHYLGKEMVQNLMVLRFANRIFGPIWNRDNIACVILTFKEPFGTEGRGGYFDEFGIIRDVMQNHLLQMLCLVAMEKPATTGSDDVRDEKVKVLKCISEVETDNVVLGQYVGNPNGEGEAANGYLDDPTVPHGSTTATFAAAVLYVENERWDGVPFILRCGKALNERKAEVRLQFRDVAGDIFHQQCKRNELVIRVQPNEAVYTKMMTKKPGMFFNPEESELDLTYGNRYKNVKLPDAYERLILDVFCGSQMHFVRSDELREAWRIFTPLLHKIDREKPQPIPYVYGSRGPTEADELMKRVGFQYEGTYKWVNPHKL

SEQ ID NO: 61 - protein, 515 aa, synthetic construct
MAEQVALSQTQTCGILWEELCQSYSFHQSDTHIFIIMGASGDLAKRNIYPTIWWLFQDGLLPKDTFIVGYTDSHFTVANIRKQSEPFFKSTPEEEPKLEEFFAHSSYMASQYDDVASYEHLNSGMNALHQGPQANCLFYLALLPSGYRTVTKNICDTCTSQTGWNRIIVEKPFGRDLQSSNQLSNHIASLFHEDQIYRIDHYLGKEVVQNLMVLRFVNRILGPIWNRDNIACMSFTFKEPFGTEGRWSYLSESGIIWEVMQNPLLQILCLVAMEKPISTNSDNIRDDKVRVLKCISKVQVSNVVLSQYMENPTEEGEATRGYPEDPRVPHGSTTDTFAAAVLYVENERWDGVPFILRCGKALNERKAEVRLQFRDVAGDIFRQQCKRNELVIRVQPNEAVYTKMMTKKPGMFFNPEESELDLTYGNRYKNVKFPDAYERLILDVFCGSQMHFVRSDELREAWRIFTPLLHHIEREKARPIPYVYGSRGPVEADELMKRVGFQYEGTYKWVNPHKL

SEQ ID NO: 62 - protein, 235 aa, synthetic construct
MQNTTQSLVVNNQVSRWQVFTAQEALNERAVRHIEEAARNAIARQGSFSIVLAGGSTPKSVYQLLPGIETDWGKWHVYYGDDRCLPPEHEERNSLMAHEAWLKHVAIPAAQVHDIPAEQGPEAAAQAYNQILQNAGEFDLVLLGLGEDGHTASLFPGHIWDDNQAAVPVFGAPKPPPERVSISAGRLSQAREVVFFVTGAGKQEAVDNWRRGEAIPASLIKPTNGVDIFIFGVNL

SEQ ID NO: 63 - protein, 331 aa, synthetic construct
MKQTVYIASPESQQIHVWNLNHEGALTLTQVVDVPGQVQPMVVSPDKRYLYVGVRPEFRVLAYRIAPDDGALTFAAESALPGSPTHISTDHQGQFVFVGSYNAGNVSVTRLEDGLPVGVVDVVEGLDGCHSANISPDNRTLWVPALKQDRICLFTVSDDGHLVAQDPAEVTTVEGAGPRHMVFHPNEQYAYCVNELNSSVDVWELKDPHGNIECVQTLDMMPENFSDTRWAADIHITPDGRHLYACDRTASLITVFSVSEDGSVLSKEGFQPTETQPRGFNVDHSGKYLIAAGQKSHHISVYEIVGEQGLLHEKGRYAVGQGPMWVVVNAH

SEQ ID NO: 64 - protein, 249 aa, synthetic construct
MVTVGVFSERASLTHQLGEFIVKKQDEALQKKSDFKVSVSGGSLIDALYESLVADESLSSRVQWSKWQIYFSDERIVPLTDADSNYGAFKRAVLDKLPSTSQPNVYPMDESLIGSDAESNNKIAAEYERIVPQVLDLVLLGCGPDGHTCSLFPGETHRYLLNETTKRVAWCHDSPKPPSDRITFTLPVLKDAKALCFVAEGSSKQNIMHEIFDLKNDQLPTALVNKLFGEKTSWFVNEEAFGKVQTKTF

SEQ ID NO: 65 - protein, 257 aa, synthetic construct
MSVYSFSDVSLVAKALGAFVKEKSEASIKRHGVFTLALSGGSLPKVLAEGLAQQRGIEFSKWEVFFADERIVPLDDENSNYALCKKLIFDKFEGFDPKKIHTINPELLKENPIDPQNVADEYEKQLVHVFANSSTVKVPVFDLLLLGCGPDGHTCSLFPDHEVLQEDVAWVAPVTDSPKPPKDRITLTLPVVTHAQAIAFVTTGAGKKDILPIVIEDFTSKLPSALITRNNLTRTSWFVDDEASANLERSSLKVFPQ

SEQ ID NO: 66 - protein, 789 aa, synthetic construct; identical to SEQ ID NO: 54

SEQ ID NO: 67 - protein, 258 aa, synthetic construct
MAAPAPRLISVFSSPQELGASLAQLVVQQAACCLADAGARFTLGLSGGSLVSMLARELPAAAAPAGPASLARWTLGFCDERLVPFEHAESTYGLYRTHLLSKLPIFDSQVITINPALPVEEAAEDYAKKLRQAFQGDSIPVFDLLILGVGPDGHTCSLFPDHPLLQEREKIVAPISDSPKPPPQRVTLTLPVLNAARTVIYVATGEGKAAILKRILEDKEENPLPAALVQPSAGKLCWFLDEAAARLLTVPFEKHSTL

SEQ ID NO: 68 - protein, 332 aa, synthetic construct
MRIGIIGLGRMGGNIAVRLTRHGHDVVVHDRTSEVTTSVVGRCEAGRATPADTLADMAKLLEGDEHRVVWVMLPAGAITEDCVQQLGGLLGRGDIIIDGGNTYYKDDVRRSAELAEKGISYVDVGTSGGVWGLERGYCMMFGGTKETAEYIDPILSALAPGIGDVPRTPGRDEAGHDPRAEQGYLHCGPAGSGHFVKMVHNGIEYGMMQAFAEGFDIMKSKNSPILAEKDRFELNMGDIAEVWRRGSVVSSWLLDLTAEALTRSETLNEFSGEVADSGEGRWTIEAAIEEDVPAPVMTAALFTRFRSRSGNNFAEKILSAQRFGFGGHVEKK

SEQ ID NO: 69 - protein, 468 aa, synthetic construct
MFNSIGVIGLGVMGSNIALNMANKGENVAVYNYTRDLTDQLIQKLDGQSLSPYYELEDFVQSLEKPRKIFLMVTAGKPVDSVIQSLKPLLEEGDVIMDGGNSHYEDTERRYDELKEKGIGYLGVGISGGEVGALTGPSIMPGGDRDVYEKAAPILTKIAAQVGDDPCCVYIGPKGAGHFTKMVHNGIEYADMQLIAEAYTFLRETLRLPLDEIASIFETWNQGELKSYLIEITAEILRKKDEKTGQPLIDVILDKTGQKGTGKWTSMQAIDNGIPSTIITESLFARYLSSLKEERMAAQDVLAGPEAEEKHLDKDTWIEYVRQALYMGKVCAYAQGFAQYKMSSELYGWNLPLKDIALIFRGGCIIRADFLNVISEAFSEQPNLANLLIAPYFTDKLHAYQTGLRKVVCEGISTGISFPCLTTALSYYDGYRTGRSNANLLQAQRDYFGAHTYERTDMDGVFHTNWSE

SEQ ID NO: 70 - protein, 332 aa, synthetic construct
MQIGIVGLGKMGGNISVRLTRHGHDVVAYDRDPAVTAKICGQGEGGRCTPATGLADMVGKLSGRRIIWLMLPAGEVTEQAVQELGTLMGKGDIIIDGGNSFYKDDIRRAAELVKKGIDYVDVGTSGGVWGLERGYCMMYGGTKEATDHIDPILSALAPGIGDIPRTPNRDRPGFDPRAEQGYLHCGPAGSGHFVKMVHNGIEYGIMQAFAEGFDVMKSKNSTDLPEDQRFELNMADIAEVWRRGSVVSSWLLDLSASALAGNPDLSNYKGDVADSGEGRWTIEAAIEEAVPVPVITASLFTRFRSRTGNNFAEKMLSAMRFGFGGHIEGTNN

SEQ ID NO: 71 - protein, 503 aa, synthetic construct
MSTNTADIGLIGLAVMGQNLALNIADHGYTISVYNRDPEKTRKFIAHAKEHEPSAGNLKGFEDLATFVLSIKRPRKIVLLVKAGSATDVTINALIPFLEEGDIIIDGGNALWTDTIRREKELRAKGLEFIGSGVSGGETGARFGPSLMPSGTQKAWSSLEPIWRDIAAKVDPRTGNPIEGATPGNPVQGGFACTEYIGPDGAGHYVKMVHNGIEYIDMQLICEAYWLMKNLLGMQSDEIGKVFEEWNKGELSSFLIEITGDILQQKDPAGDGFLVDKIMDAAGQKGTGQWTAANALELGSPANAIAAAVFARALSTVKDERVEASTILKGPKIQQEADREKLIESIRNALYCSKICAYAQGFQLIDKAQVAYNWKLNFGEIAQIWRGGCIIRARFLQKITDAYALDAHLTNLMLDPYFTEALDEGQSSWREVVSLAVRNGIPAQAFCAALSYYDGYRSATLPANLLQAQRDYFGAHTYERVDQPRGQFFHVDWPEPGRPQLKV

SEQ ID NO: 72 - protein, 468 aa, synthetic construct
MSKQQIGVVGMAVMGRNLALNIESRGYTVSIFNRSREKTEEVIAENPGKKLVPYYTVKEFVESLETPRRILLMVKAGAGTDAAIDSLKPYLDKGDIIIDGGNTFFQDTIRRNRELSAEGFNFIGTGVSGGEEGALKGPSIMPGGQKEAYELVAPILTKIAAVAEDGEPCVTYIGADGAGHYVKMVHNGIEYGDMQLIAEAYSLLKGGLNLTNEELAQTFTEWNNGELSSYLIDITKDIFTKKDEDGNYLVDVILDEAANKGTGKWTSQSALDLGEPLSLITESVFARYISSLKDQRVAASKVLSGPQAQPAGDKAEFIEKVRRALYLGKIVSYAQGFSQLRAASEEYNWDLNYGEIAKIFRAGCIIRAQFLQKITDAYAENPQIANLLLAPYFKQIADDYQQALRDVVAYAVQNGIPVPTFSAAVAYYDSYRAAVLPANLIQAQRDYFGAHTYKRIDKEGVFHTEWLD

SEQ ID NO: 73 - protein, 489 aa, synthetic construct
MSADFGLIGLAVMGQNLILNAADHGFTVCAYNRTQSKVDHFLANEAKGKSIIGATSIEDFISKLKRPRKVMLLVKAGAPVDALINQIVPLLEKGDIIIDGGNSHFPDSNRRYEELKKKGILFVGSGVSGGEEGARYGPSLMPGGSEEAWPHIKNIFQSISAKSDGEPCCEWVGPAGAGHYVKMVHNGIEYGDMQLICEAYDIMKRLGGFTDKEISDVFAKWNNGVLDSFLVEITRDILKFDDVDGKPLVEKIMDTAGQKGTGKWTAINALDLGMPVTLIGEAVFARCLSALKNERIRASKVLPGPEVPKDAVKDREQFVDDLEQALYASKIISYAQGFMLIREAAATYGWKLNNPAIALMWRGGCIIRSVFLGQITKAYREEPDLENLLFNKFFADAVTKAQSGWRKSIALATTYGIPTPAFSTALSFYDGYRSERLPANLLQAQRDYFGAHTFRVLPECASDNLPVDKDIHINWTGHGGNVSSSTYQA

SEQ ID NO: 74 - protein, 492 aa, synthetic construct
MSQKEVADFGLIGLAVMGQNLILNGADKGFTVCCYNRTTSRVDEFLANEAKGKSIVGAHSLEEFVSKLKKPRVCILLVKAGKPVDYLIEGLAPLLEKGDIIVDGGNSHYPDTTRRCEELAKKGILFVGSGVSGGEEGARYGPSLMPGGNPAAWPRIKPIFQTLAAKAGNNEPCCDWVGEQGAGHYVKMVHNGIEYGDMQLICETYDIMKRGLGMSCDEIADVFEKWNTGKLDSFLIEITRDVLRYKADDGKPLVEKILDAAGQKGTGKWTAQNALEMGTPVSLITEAVFARCLSSLKSERVRASKKLTGPNTKFTGDKKQLIDDLEDALYASKIISYAQGFMLMREAAKEYGWKLNNAGIALMWRGGCIIRSVFLKDITEAFREDPNLESILFHPFFTNGVEKAQAGWRRVVAQAAMLGIPVPATSTGLSFYDGYRSAVLPANLLQAQRDYFGAHTFRVLPEAADKSLPADKDIHINWTGHGGNISATTYDA

SEQ ID NO: 75 - protein, 483 aa, synthetic construct
MAQADIALIGLAVMGQNLILNMNDHGFVVCAFNRTVSKVDDFLAKEAKGTKVIGAKSLKDMVSKLKKPRRVILLVKAGQAVDDFIEKLVPLLDTGDIIIDGGNSEYRDTTRRCQDLKAKGILFVGSGVSGGEEGARYGPSLMPGGNKEAWPHIKTIFQAIAAKVGTGEPCCDWVGDEGAGHFVKMVHNGIEYGDMQLICEAYHLMKDVLGMRHEEMAQAFEDWNKTELDSFLIEITANILKFQDTDGKELLPKIRDSAGQKGTGKWTAISALEYGMPVTLIGEAVFARCLSSLKEERVQASRKLKGPKMVQLEGSKQAFLEDVRKALYASKIISYAQGFMLLRQAATEFGWTLNYGGIALMWRGGCIIRSVFLGKIKDAFERNPELQNLLLDDFFKSAVDDCQDSWRRVISTGVQAGIPMPCFTTALSFYDGYRHEMLPANLIQAQRDYFGAHTYELLSKPGEFIHTNWTGHGGSVSSSSYNA

SEQ ID NO: 76 - protein, 250 aa, synthetic construct
IEITANILKFQDADGKHLLPKIRDSAGQKGTGKWTAISALEYGVPVTLIGEAVFARCLSSLKDERVQASKKLKGPQKIQFSGDKKSFLEDIRKALYASKIISYTQGFMLLRQAAAEFGWSSTTEHRLMWRGGCIIRSVFLGKIKDAFDRNPGLQNLLLDDFFKSAVEDCQDSWRRAVSTGVQTGIPMPCFTTALSFYDGYRHEMLPANLIQAQRDYFGAHTYELLAKPGHFVHTNWTGHGGSVSSSSYNA

SEQ ID NO: 77 - protein, 258 aa, synthetic construct
MQIERAGALVTGGASGLGLATARRLAAGGALVTILDLPTSRGAEIAAELGGVFAPADVTSVPEVRAAVAEASALAPLRVVVACAGIATPGKVLDREGSPTPLEDFERVVRINLVGTYNVISQAAAAMVANEPTETDSDASDERGVIVTTASVAAFDGQIGQPAYAASKGGVHAMTLPIARELARYGIRVVTIAPGIMETPLLQALPQAAQDSLGGQVPFPARLGRPEEFAALVAHIAENGYLNGETIRLDGAIRMAPK

SEQ ID NO: 78 - protein, 254 aa, synthetic construct
MELKGLSVAITGGASGLGLATARRVLDAGGTVTLVDLPGSPGADVAKSLGDGATFAAADVTDAEQFAAALDVAHERGGLRGLVHCAGAGRKMRVLDKDGKAGSLEDFEFVIRLNLIGSFNALRLGAERMAALEPVDGERGAIVMTASVAAFEGQIGQINYSASKAGIVGMTVVAARDLASKNIRVNTIAPGIMDTPLLARLRDDVRASLEKTVPNPARLGRPDEFGQLATSILENGYLNGETIRLDGAIRMAPR

SEQ ID NO: 79 - protein, 252 aa, synthetic construct
MQIAQQVFIVTGGASGLGAATARRLAGMGGKVLIADVQDDAGQALAHAVQGRYVHCDVTREDDAAQAVALALELGPLRGLVNCAGVAPASRTLGKEGPHPLDVFVRTITINLVGSFNMARLAAAAMAKQEALDDGERGVVVHTASVAAYDGQIGQTAYAASKAGIVGMTLPMARDLARDGIRVMTIAPGIFETPMLMGMPEAVRAALGAAVPFPSRLGRPDEFAMLVEAIVTNPMLNGETIRLDGAIRMQPK

SEQ ID NO: 80 - protein, 604 aa, synthetic construct
MTQTLIEVTERIRERSAPTRKAYLQRIDQIINRTRGADRLGCANVAHAFAALPNNDKFRVVAEKAPHIGIVTAYNDMLSAHQPYENYPNIIRDEARKHGATVQVAGGVPAMCDGITQGEPGMELSLFSRDTIAMSTAVSLSHDVFDAALMLGVCDKIVPGLLIGALHFGHLPTVFVPAGPMATGIDNTTKSKVREKYAQGLVGREELLASESAAYHGAGTCTFFGTANSNQMLIEAMGLHVPGAAFVHPHDDMREMLTRESVKTVLSITKGQRFTPIGQMVDERVIVNAIVALLATGGSTNHLIHWVAVARAAGIIIDWSDFSKLSQNTPLLARVYPNGTADVNQFQAAGGPSFVIRELVDAGYMHGDVNSVVIGGLRDFGKKPVKSDDELIWVDLPKESPDETIVRNASKPFSASGGLRLLTGNLGRSVIKSSAVPEDRQIIEAPAIVFNGQEELLAAFERGELEKDFIAVVRFQGPRANGMPELHKLTPPLSVLQGKGFRVAIVTDGRMSGASGKVPAAIHLSPEGVAGGAICKIRTGDMIRLNAIVGTLNALVDDEEWQARTVAVMTEAQRNNNGHGIGRELFGGMRKNVHSAEEGAVTWL

SEQ ID NO: 81 - protein, 624 aa, synthetic construct
MSNAFSDNSRLNSTFSSTPLMTQTLIEVTERIRERSAPTRKAYLQRIDQIINRTRGPDRLGCANVAHAFAALPSNDKFRVVAEKAPHIGIVTAYNDMLSAHQPYETYPSIIRDEARKHGATVQVAGGVPAMCDGITQGEPGMELSLFSRDTIAMSTAISLSHDVFDAALMLGVCDKIVPGLLIGALHFGHLPTLFVPAGPMATGIDNTTKSKVREKYAQGLVGRDELLASESAAYHGAGTCTFFGTANSNQMLIEAMGLHVPGAAFVHPHDDMRELLTREAVKTVLSITKGQRFTPIGKMVDERVIVNAIVALLATGGSTNHLIHWVAVARAAGIIIDWSDFSKLSQNTPLLARVYPNGTADVNQFQAAGGPSFVIRELIEGGYMHGDVTSVVLGGLRDFCKKPVKSDDGLIWVDLPKESPDETIVRNVSKPFSATGGLRLLTGNLGRSVIKSSAVPEDRQIIEAPAIVFNGQEELLAAFERGELEKDFIAVVRFQGPRANGMPELHKLTPPLSVLQGKGFRVAIVTDGRMSGASGKVPAAIHLSPEAVAGGAIGKIRTGDMIRLNAIVGTLNALVDDEEWQARPVAVMTEAQRNNNSHGIGRELFGGMRKNVHSAEEGAVTWL

SEQ ID NO: 82 - protein, 603 aa, synthetic construct
MNPQLLRVTNRIIERSRETRSAYLARIEQAKTSTVHRSQLACGNLAHGFAACQPEDKASLKSMLRNNIAIITSYNDMLSAHQPYEHYPEIIRKALHEANAVGQVAGGVPAMCDGVTQGQDGMELSLLSREVIAMSAAVGLSHNMFDGALFLGVCDKIVPGLTMAALSFGHLPAVFVPSGPMASGLPNKEKVRIRQLYAEGKVDRMALLESEAASYHAPGTCTFYGTANTNQMVVEFMGMQLPGSSFVHPDSPLRDALTAAAARQVTRMTGNGNEWMPIGKMIDEKVVVNGIVALLATGGSTNHTMHLVAMARAAGIQINWDDFSDLSDVVPLMARLYPNGPADINHFQAAGGVPVLVRELLKAGLLHEDVNTVAGFGLSRYTLEPWLNNGELDWREGAEKSLDSNVIASFEQPFSHHGGTKVLSGNLGRAVMKTSAVPVENQVIEAPAVVFESQHDVMPAFEAGLLDRDCVVVVRHQGPKANGMPELHKLMPPLGVLLDRCFKIALVTDGRLSGASGKVPSAIHVTPEAYDGGLLAKVRDGDIIRVNGQTGELTLLVDEAELAAREPHIPDLSASRVGTGRELFSALREKLSGAEQGATCITF

SEQ ID NO: 83 - protein, 161 aa, synthetic construct
MSSYTPSSESGTDDAVEDGTLSGADVFDTDDCVLSGADAVDDWPLSGADVAPRLGPGRTLRNVNVTGAAPYDDEGDSARLVLKLVVVLVIVLGIKLLLGRTSSPRLWLAINVFFDFGVYAYSEFSELPPCSLSFSPLLLRRLFPRTLAGLSDSAVDPTPTL

SEQ ID NO: 84 - protein, 130 aa, synthetic construct
MRFSLSIATGLAAAGLVRATREFTLILHVTVRPKMLNQTPPALEARRVARDWLTRPTMFVPVQLRTAGDTSHLQLGFWNLTYRGDLGALQLDLKTNYTTAVHGLGQRAGHLRRRWIRSSLTDIRDAALVA

SEQ ID NO: 85 - protein, 209 aa, synthetic construct
MSTLDLANHGPVIPVIVINKVEDAVPMAEALLEGGIKVLEVTLRTPVALQAMEAIAKAVPDAIVGAGTVRNIKDAQNCKDVGCQFAVSPGYTSELGRAAREMGLPLLPGVSTGSEIMQANADDYYFLKLFPAVAVGGINLLKGFAGPFGDVKFCPTGGLTVESAPQFLALPNVVVCGGTWLTPGDAVARKDWAHITKLAREASAIKAAA

SEQ ID NO: 86 - protein, 214 aa, synthetic construct
MAVNNEKLTALQVMLDASVIPVIVLNDVAHAVPMAKALVAGGIRMLEITLRTSVALDCMRAIAAEVPEAVIGAGTIRSAADAKAALAAGARFGVSPGYTTTVGKTCQDIGLPLLPGVATGSEIMIAQEDGFTELKFFPAMQAGGPNLLKAWAGPFTDIKFCPTGGVSLENAPTLLALPNVVVVGGSWLTPADVMARGEWSRITEMASEACKLAR

SEQ ID NO: 87 - protein, 213 aa, synthetic construct
MKNWKTSAESILTTGPVVPVIVVKKLEHAVPMAKALVAGGVRVLEVTLRTECAVDAIRAIAKEVPEAIVGAGTVLNPQQLAEVTEAGAQFAISPGLTEPLLKAATEGTIPLIPGISTVSELMLGMDYGLKEFKFFPAEANGGVKALQAIAGPFSQVRFCPTGGISPANYRDYLALKSVLCIGGSWLVPADALEAGDYDRITKLAREAVEGAKL

SEQ ID NO: 88 - protein, 196 aa, synthetic construct
MESKVVENRLKEAKLIAVIRSKDKQEACQQIESLLDKGIRAVEVTYTTPGASDIIESFRNREDILIGAGTVISAQQAGEAAKAGAQFIVSPGFSADLAEHLSFVKTHYIPGVLTPSEIMEALTFGFTTLKLFPSGVFGIPFMKNLAGPFPQVTFIPTGGIHPSEVPDWLRAGAGAVGVGSQLGSCSKEDLQAVFQV

SEQ ID NO: 89 - protein, 779 aa, synthetic construct
MHPNLLRVTSRIIERSRPTREAYLARIEKARSNTVHRSELACGNLAHGFAACQPDDKAALKSMLRNNIAIITSYNDMLSAHQPYEHYPEQIRKALHSVGAVGQVAGGVPAMCDGVTQGQDGMELSLLSREVIAMSTAVGLSHNMFDGALYLGVCDKIVPGLTMAALSFGHLPALFVPSGPMASGLPNKEKVRIRQLYAEGKVDRLALLEAEAASYHAPGTCTFYGTANTNQMVVEFMGMQLPGSSFVQPDAELRGALTDAAARQVTRLTGNGNEWMPLGKMIDEKVVVNGIVALLATGGSTNHTMHLVAMARAAGIIINWDDFSDISEIVPLLARLYPNGPADINHFQAAGGVPVLMRELLKGGLLHEDVNTVAGFGLHHYTMEPWLDNGQLAWREGASQPLDSDVIATMEKPFSRHGGTKVLSGNLGRAVMKTSAVPVENQVIEAPAVIFESQHDVLPAFEAGKLDRDCVVVVRHQGPKANGMPELHKLMPPLGVLLDRCFKIALVTDGRLSGASGKVPSAIHVTPEAYDGGLLAKVQDGDMIRVNGQTGELTLLVDEAVLAARTAYHPDLSAERILKTGPVVPVIVVNKLEHAVPMAKALVAGGVRVLEVTLRTACAIDAIRAIAKEVPEAIIGAGTVLNPQQLAEVTEAGAQFAISPGLTEPLLKAATEGTIPLIPGISTVSELMLGMDYGLKEFKFFPAEANGGTKALQAIAGPFSQVRFCPTGGISPANYRDYLALKSVLCIGGSWLVPADALEAGDYDRITKLAREAVEGAKL

SEQ ID NO: 90 - protein, 288 aa, synthetic construct
MEIISPIITPFDKQGKVNVDALKTHAKNLLEKGIDAIFVNGTTGLGPALSKDEKRQNLNALYDVTHKLIFQVGSLNLNDVMELVKFSNEMDILGVSSHSPYYFPRLPEKFLAKYYEEIARISSHSLYIYNYPAATGYDIPPSILKSLPVKGIKDTNQDLAHSLEYKLNLPGVKVYNGSNTLIYYSLLSLDGVVASFTNFIPEVIVKQRDLIKQGKLDDALRLQELINRLADILRKYGSISAIYVLVNEFQGYDVGYPRPPIFPLTDEEALSLKREIEPLKRKIQELVH

SEQ ID NO: 91 - protein, 215 aa, synthetic construct
MSHHPARRIRETGLIAIIRGTDADTAIETVEALTRGGVSTVEITANTDGVLGMLRDVSASFTADEVTIGAGTVLDSETARAALLAGAEYLVTPTFDEGVIRTGNRYGAPSMVGIATPTEAVNAYEAGAEMVKVFPAGTLGPEFVSALGGPLGHIPTVPTGGVALDTVDEFFDAGATAVGVGSAIVDNDAVSRGDFATIETNARSFVEAVERARRD

SEQ ID NO: 92 - protein, 250 aa, synthetic construct
MRRKLVVGNWKMNGNLAQNKRLLEALVRGLQDVEHVDIAVCVPYPYLFQAQKILSGTNIAWGAQNVAKHENGAYTGEVSAAMLKEFGASYVIVGHSERSDAYCESNANIAEKFAIAKHYGITPIFCVGETLQERESGVMEYAIANQLDAVLSVSGGALLDQAVIAYEPVWAIGTNRTATPEQARAAHSFIRERIAAMHPGAAESVRIIYGGSVNPRNAAQLLSMPDIDGGLIGRCSLDADDFERICRAAC

SEQ ID NO: 93 - protein, 255 aa, synthetic construct
MRHPLVMGNWKLNGSRHMVHELVSNLRKELAGVAGCAVAIAPPEMYIDMAKREAEGSHIMLGAQNVDLNLSGAFTGETSAAMLKDIGAQYIIIGHSERRTYHKESDELIAKKFAVLKEQGLTPVLCIGETEAENEAGKTEEVCARQIDAVLKTQGAAAFEGAVIAYEPVWAIGTGKSATPAQAQAVHKFIRDHIAKVDANIAEQVIIQYGGSVNASNAAELFAQPDIDGALVGGASLKADAFAVIVKAAEAAKQA

SEQ ID NO: 94 - protein, 248 aa, synthetic construct
MARTFFVGGNFKLNGSKQSIKEIVERLNTASIPENVEVVICPPATYLDYSVSLVKKPQVTVGAQNAYLKASGAFTGENSVDQIKDVGAKWVILGHSERRSYFHEDDKFIADKTKFALGQGVGVILCIGETLEEKKAGKTLDVVERQLNAVLEEVKDWTNVVVAYEPVWAIGTGLAATPEDAQDIHASIRKFLASKLGDKAASELRILYGGSANGSNAVTFKDKADVDGFLVGGASLKPEFVDIINSRN

SEQ ID NO: 95 - protein, 249 aa, synthetic construct
MARKFFVGGNFKMNGSLESMKTIIEGLNTTKLNVGDVETVIFPQNMYLITTRQQVKKDIGVGAQNVFDKKNGAYTGENSAQSLIDAGITYTLTGHSERRTIFKESDEFVADKTKFALEQGLTVVACIGETLAEREANETINVVVRQLNAIADKVQNWSKIVIAYEPVWAIGTGKTATPEQAQEVHAEIRKWATNKLGASVAEGLRVIYGGSVNGGNCKEFLKFHDIDGFLVGGASLKPEFHNIVNVHSL

SEQ ID NO: 96 - protein, 249 aa, synthetic construct
MAPSRKFFVGGNWKMNGRKKCLGELICTLNAAKLPADTEVVCAPPTAYIDFARQKLDPKIAVAAQNCYKVTNGAFTGEISPGMIKDLGATWVVLGHSERRHIFGESDELIGQKVNHALSEGLGVIACIGEKLDEREAGITEKVVFEQTKAIADNVKDWCKVVLAYEPVWAIGTGKTATPQQAQEVHEKLRGWLKCNVSEGVAQCTRIIYGGSVTGATCKELASQPDVDGFLVGGASLKPEFVDIINAKQ

SEQ ID NO: 97 - protein, 248 aa, synthetic construct
MAPRKFFVGGNWKMNGDKKSLGELIHTLNGAKLSADTEVVCGAPSIYLDFARQKLDAKIGVAAQNCYKVPKGAFTGEISPAMIKDIGAAWVILGHSERRHVFGESDELIGQKVAHALAEGLGVIACIGEKLDEREAGITEKVVFEQTKAIADNVKDWSKVVLAYEPVWAIGTGKTATPQQAQEVHEKLRGWLKSHVSDAVAQSTRIIYGGSVTGGNCKELASQHDVDGFLVGGASLKPEFVDIINAKH

SEQ ID NO: 98 - protein, 309 aa, synthetic construct
MVRIYTLTLAPSLDSATITPQIYPEGKLRCTAPVFEPGGGGINVARAIAHLGGSATAIFPAGGATGEHLVSLLADENVPVATVEAKDWTRQNLHVHVEASGEQYRFVMPGAALNEDEFRQLEEQVLEIESGAILVISGSLPPGVKLEKLTQLISAAQKQGIRCIVDSSGEALSAALAIGNIELVKPNQKELSALVNRELTQPDDVRKAAQEIVNSGKAKRVVVSLGPQGALGVDSENCIQVVPPPVKSQSTVGAGDSMVGAMTLKLAENASLEEMVRFGVAAGSAATLNQGTRLCSHDDTQKIYAYLSR

SEQ ID NO: 99 - protein, 322 aa, synthetic construct
MNKIAVLTSGGDAPGMNAAIRAVVRRGIFKGLDVYGVKNGYKGLMNGNFVSMNLGSVGDIIHRGGTILQTTRCKEFKTAEGQQQALAQLKKEGIDGLIVIGGDGTFEGARKLTAQEFPTIGIPATIDNDIAGTEYTIGFDTAVNTAVEAIDKIRDTAASHDRIYVVEVMGRNAGDIALWAGMCAGAESIIIPEADHDVEDVIDRIKQGYQRGKTHSIIVVAEGAFNGVGAIEIGRAIKEKTGFDTKVTILGHIQRGGSPSAYDRMMSSQMGAKAVDLLVEGKKGLMVGLKNGQLIHTPFEEAAKDKHTVDLSIYHLARSLSL

SEQ ID NO: 100 - protein, 987 aa, synthetic construct
MQSQDSCYGVAFRSIITNDEALFKKTIHFYHTLGFATVKDFNKFKHGENSLLSSGTSQDSLREVWLESFKLSEVDASGFRIPQQEATNKAQSQGALLKIRLVMSAPIDETFDTNETATITYFSTDLNKIVEKFPKQAEKLSDTLVFLKDPMGNNITFSGLANATDSAPTSKDAFLEATSEDEIISRASSDASDLLRQTLGSSQKKKKIAVMTSGGDSPGMNAAVRAVVRTGIHFGCDVFAVYEGYEGLLRGGKYLKKMAWEDVRGWLSEGGTLIGTARSMEFRKREGRRQAAGNLISQGIDALVVCGGDGSLTGADLFRHEWPSLVDELVAEGRFTKEEVAPYKNLSIVGLVGSIDNDMSGTDSTIGAYSALERICEMVDYIDATAKSHSRAFVVEVMGRHCGWLALMAGIATGADYIFIPERAVPHGKWQDELKEVCQRHRSKGRRNNTIIVAEGALDDQLNPVTANDVKDALIELGLDTKVTILGHVQRGGTAVAHDRWLATLQGVDAVKAVLEFTPETPSPLIGILENKIIRMPLVESVKLTKSVATAIENKDFDKAISLRDTEFIELYENFLSTTVKDDGSELLPVSDRLNIGIVHVGAPSAALNAATRAATLYCLSHGHKPYAIMNGFSGLIQTGEVKELSWIDVENWHNLGGSEIGTNRSVASEDLGTIAYYFQKNKLDGLIILGGFEGFRSLKQLRDGRTQHPIFNIPMCLIPATVSNNVPGTEYSLGVDTCLNALVNYTDDIKQSASATRRRVFVCEVQGGHSGYIASFTGLITGAVSVYTPEKKIDLASIREDITLLKENFRHDKGENRNGKLLVRNEQASSVYSTQLLADIISEASKGKFGVRTAIPGHVQQGGVPSSKDRVTASRFAVKCIKFIEQWNKKNEASPNTDAKVLRFKFDTHGEKVPTVEHEDDSAAVICVNGSHVSFKPIANLWENETNVELRKGFEVHWAEYNKIGDILSGRLKLRAEVAALAAENK

SEQ ID NO: 101 - protein, 942 aa, synthetic construct
MSGETVHGISCYSVVANTEDTYNQTLDFYQKLGFKKVASFGTSDSDNARVCNESLREDWMHVAGNNSAESVTIKFRLVPGELSLSPAAEDSEWRGQKSSLVFYYPNLLDLLKQLSADAIKYQAFPNEKKPDEVYVEDPLGNLIGFSDRYNPFAHANLKKSEESGAASNLESGLATPVVETLKKATTSDKPAGVKKKIAVMTSGGDSPGMNAVVRAVARIAIHRGCDAFAIYEGYEGLVQGGDMIKQLQWGDVRGWLAEGGTLIGTARCMAFRERPGRLRAAKNLISAGIDSIIVCGGDGSLTGADIFRSDWPGLVKELEDTKAITPEQAKLYRHLTIVGLVGSIDNDMSSTDVTIGAFSSLHRICEAVDSISSTAISHSRAFIVEVMGRHCGWLAVLAALATGADFVFIPERPAEVGKWQDELCNSLSSVRKLGKRKSIVIVAEGAIDSELNHISPEDIKNLLVERLHLDTRVTTLGHVQRGGIPCAYDRMLATLQGVDAVDAVLASTPDTPSPMIAINGNKINRKPLMEAVKLTHEVADAIEKKQFAHAMELRDPEFADYLHTWEGTTFIEDESHFVPKDERMRVAIIHVGAPAGGMNSATRAAVRYCLNRGHTPLAIDNGFSGFLRHDSIHELSWIDVDEWCIRGGSEIGTNRDTPDLDMGFTAFKFQQHKIDALIIIGGFEAFTALSQLESARVNYPSFRIPMAIIPATISNNVPGTEFSLGCDTCLNAVMEYCDTIKQSASASRRRVFVCEVQGGRSGYIATVGGLITGASAIYTPEDGISLDMLRKDIDHLKATFALEAGRNRAGQLILRNECASKVYTTEVIGNIISEEAHKRFSARTAVPGHVQQGGNPTPMDRARAARLAMRAIRFFETCRANDLGNDPSSAVVIGIRGTGVSFSSVADVENNETEIEMRRPKNAWWRDMHNLVNILAGKTFAD

SEQ ID NO: 102 - protein, 780 aa, synthetic construct
MATVDLEKLRMSGAGKAIGVLTSGGDAQGMNAAVRAVTRMGIYVGAKVFLIYEGYEGLVEGGENIKPANWLSVSNIIQLGGTIIGSARCKAFTTREGRLAAAYNLLQHGITNLCVIGGDGSLTGANIFRNEWGSLLEELVKEGKISESTAQNYAHLTIAGLVGSIDNDFCGTDMTIGTDSALHRIMEVIDAITTTAQSHQRTFVLEVMGRHCGYLALVSALASGADWLFIPEAPPEDGWENFMCERLGETRSRGSRLNIIIIAEGAIDRHGKPISSSYVKDLVVQRLGFDTRVTVLGHVQRGGTPSAFDRILSSKMGMEAVMALLEATPDTPACVVSLSGNQSVRLPLMECVQVTKDVQKAMDEERFDEAIQLRGRSFENNWKIYKLLAHQKVSKEKSNFSLAILNVGAPAAGMNAAVRSAVRTGISEGHTVYIVHDGFEGLAKGQVQEVGWHDVAGWLGRGGSMLGTKRTLPKPHLEAIVENLRTYNIHALLVIGGFEAYEGVLQLVEARGRYEELCIVMCVIPATISNNVPGTDFSLGSDTAVNAAMESCDRIKQSASGTKRRVFIVETMGGYCGYLATVTGIAVGADAAYVFEDPFNIHDLKANVEHMTEKMKTDIQRGLVLRNEKCHEHYTTEFLYNLYSSEGRGVFDCRTNVLGHLQQGGAPTPFDRNYGTKLGVKAMLWVSEKLRDVYRKGRVFANAPDSACVIGLRKKVVAFSPVTELKKETDFEHRMPREQWWLNLRLMLKMLAHYRISMADYVSGELEHVTRRTLSIDKGF

SEQ ID NO: 103 - protein, 779 aa, synthetic construct
MTHEHHAAKTLGIGKAIAVLTSGGDAQGMNAAVRAVVRVGIYTGARVFFVHEGYQGLVDGGDNIREATWESVSMMLQLGGTVIGSARCKDFREREGRLRAAHNLVKRGITNLCVIGGDGSLTGADTFRSEWSDLLSDLQKSGKITAEEATKSSYLNIVGLVGSIDNDFCGTDMTIGTDSALHRIIEIVDAITTTAQSHQRTFVLEVMGRHCGYLALVTSLSCGADWVFIPECPPDDDWEEHLCRRLSETRNRGSRLNIIIVAEGAIDKNGKPITSEDIKNLVVKRLGYDTRVTVLGHVQRGGTPSAFDRILGSRMGVEAVMALLEGTPDTPACVVSLSGNQAVRLPLMECVQVTKDVTRAMDERRFDEALKLRGRSFMNNWEVYKLLAHVRPPKSKSGSHTVAVMNVGAPAAGMNAAVRSTVRIGLIQGNRMLVVHDGFEGLAKGQIEEAGWSYVGGWTGQGGSKLGTKRTLPKKSFEQISANITKFNIQGLVIIGGFEAYTGGLELMEGRKQYDELCIPFVVIPATVSNNVPGSDFSVGADTALNTICMTCDRIKQSAAGTKRRVFIIETMGGYCGYLATMAGLAAGADAAYIFEDPFTIRDLQVNVEHLVQKMKTTVKRGLVLRNEKCNENYTTDFIFNLYSEEGKGIFDSRKNVLGHMQQGGSPTPFDRNFATKMGAKAMNWMSGKIKESYRNGRIFANSPDSGCVLGMRKRALVFQPVTELKEQTDFEHRIPKEQWWLKLRPILKILAKYEIDLDTSEHAHLEHISRKRSGEANV

SEQ ID NO: 104 - protein, 413 aa, synthetic construct
MGEDLVLGLGGTVDYEIRWDAAVLSALAREHGIHLGELTTTTPIIDERALVVTVLAFLATGGGGERFVLSSEIVERFASHFDVETTLGGTGVRAGIALDRIGVPTVQHLVSIDDNVRRLLPTSMRIVSSATQDTLDPHLIVQYPEGTTVELVDATVTASASNRLIFANDAPNREMAIAAGLGEALARAAAFLVSGFNTMQDAAMLERRLDDLTAAMRHLPADALVYYEDAGFYQRELSSLVRARLLDRIDVYGMNEDELQEYLARPVDLLSPDDVVAALAEVHDLIPARALVVHTKYWAIAVGPHAARHRAGLESAVRTAATRYRLGDACTAADLEDTARLPRHAGGAAVVAAAESRRGATGVPAFLVDTAHPTTIGLGDTFVGGFLAAVPAAARLATAVALERALDATSPVR

SEQ ID NO: 105 - protein, 413 aa, synthetic construct; identical to SEQ ID NO: 104

SEQ ID NO: 106 - protein, 345 aa, synthetic construct
MSARLMQFRAGRAFRQGETNTVVPEAGRGLVYLQEEDGLLHFCYKNLETNQVDEDLIIFPGDASFANATPDRVHVLRFNSSSARHFFWHQDPQLDQAEFEQRGRRVNELIGAEPVDVAAPAAPAAGNMDVEPSSGDVAMSDAPASSTASDSTAFETPAVARTVPDSQTAAAAAAAPPGAPRKLGQAEQLAQLQSILAGLGGTSNTNAASLLQSATHSGGVPEFTLPDVLTPSAATSLIASLPDSSLSHLSSFLPTRVPTLPLSTPAEQRASLIRAVGSPEFRRALASLERALRTGATGPLVQGLGMQARAAHGTQEFLEEVQRQADQEREREGGGAGASEPGSAP

SEQ ID NO: 107 - protein, 409 aa, synthetic construct
MNKPKKVAILTAGGLAPCLNSAIGSLIERYTEIDPSIEIICYRGGYKGLLLGDSYPVTAEVRKKAGVLQRFGGSVIGNSRVKLTNVKDCVKRGLVKEGEDPQKVAADQLVKDGVDILHTIGGDDTNTAAADLAAFLARNNYGLTVIGLPKTVDNDVFPIKQSLGAWTAAEQGARYFMNVVAENNANPRMLIVHEVMGRNCGWLTAATAQEYRKLLDRAEWLPELGLTRESYEVHAVFVPEMAIDLEAEAKRLREVMDKVDCVNIFVSEGAGVEAIVAEMQAKGQEVPRDAFGHIKLDAVNPGKWFGEQFAQMIGAEKTLVQKSGYFARASASNVDDMRLIKSCADLAVECAFRRESGVIGHDEDNGNVLRAIEFPRIKGGKPFNIDTDWFNSMLSEIGQPKGGKVEVSH

SEQ ID NO: 108 - protein, 342 aa, synthetic construct
MKVGVLTGGGDCPGLNAVIRAVVRKGVQEYGYDFTGFRDGWRGPLEGDTVPLDIPAVRGILPRGGTVLGSSRTNPLKQRDGIRRIKDNLAALGVEALITIGGEDTLGVATRLADEYGVPCVGVPKTIDNDLSATDYTFGFDTAVGIATEAIDRLHTTAESHMRVLVVEVMGRHAGWIALHSGLAGGANVILIPEQRFDVEQVCSWVTSRFRASYAPIVVVAEGAMPRDGDMVLKDESLDSYGHVRLSGVGEWLAKQIEKRTGNEARTTVLGHVQRGGTPSAFDRWLATRFGLHAVDCVHDGDFGKMVALRGTDIVRVPIAEATARLKTVDPALYEEVGVFFG

SEQ ID NO: 109 - protein, 419 aa, synthetic construct
MSKKIKNAFYAQSGGVTAVINASACGVIETARKHPDKIGKVYAGRNGIIGALTEDLIDTSKESDAAIAALRSTPSGAFGSCRYKLKSLETNRREYERLIEVFRAHDIGYFFYNGGGDSADTCYKISQLSETMGYPVQAIHVPKTVDNDLPITDNCPGFGSVAKYIAISTLEASFDVRSMCKTSTKIFVIEVMGRHAGWIAAAGGLVEDYGFPVVILFPEIEFDPEKFLARVDKMVKKHGHCTVVVSEGCHYPDGKFIAEQGIKDVFGHAQLGGAAPIVANMIKNALGHRFHWAVADYLQRAARHIASRTDVKQAYELGKAAVDLALKGKNSVMPAIIRVSDEPYKYRIGHAELKDVANVEKFMPLDFISKDGFGITEKCKRYLRPLIQGEDYPKYEDGLPVYVSLKNMPVERRLPEFSL

SEQ ID NO: 110 - protein, 279 aa, synthetic construct
VSLRQLLDHAAENGYGLPAFNVNNMEQIHAIMQAADAVDSPVILQGSAGARKYAGESFLRHMIAAAVEAYPHIPLVMHQDHGASPAVCIQAIRSGFSSVMMDGSLKEDMKTPASYDYNVDVTRKVVDMAHAVGVSVEGELGCLGSLETGMAGEEDGHGAEGVLDHSALLTDPEEAADFVKKTGVDALAIAIGTSHGAYKFSRPPTGETLAINRIKEIHARIPNTHLVMHGSSSVPQEWLKIINANGGQIPETYGVPVEEIVEGIKHGVRKVNIDTDLRL

SEQ ID NO: 111 - protein, 285 aa, synthetic construct
MPLVSMTEMLNTAKEKGYAVGQFNLNNLEFTQAILQAAEEEKSPVILGVSEGAGRYMGGFKTVVAMVKALMEEYKVTVPVAIHLDHGSSFESCAKAIHAGFTSVMIDASHHPFEENVATTAKVVELAHFHGVSVEAELGTVGGQEDDVIAEGVIYADPKECQELVERTGIDCLAPALGSVHGPYKGEPNLGFKEMEEIGKSTGLPLVLHGGTGIPTADIKKSISLGTAKINVNTENQISSAKAVRETLAAKPDEYDPRKYLGPAREAIKETVIGKMREFGSSNQA

SEQ ID NO: 112 - protein, 359 aa, synthetic construct
MGVEQILKRKTGVIVGEDVHNLFTYAKEHKFAIPAINVTSSSTAVAALEAARDSKSPIILQTSNGGAAYFAGKGISNEGQNASIKGAIAAAHYIRSIAPAYGIPVVLHSDHCAKKLLPWFDGMLEADEAYFKEHGEPLFSSHMLDLSEETDEENISTCVKYFKRMAAMDQWLEMEIGITGGEEDGVNNENADKEDLYTKPEQVYNVYKALHPISPNFSIAAAFGNCHGLYAGDIALRPEILAEHQKYTREQVGCKEEKPLFLVFHGGSGSTVQEFHTGIDNGVVKVNLDTDCQYAYLTGIRDYVLNKKDYIMSPVGNPEGPEKPNKKFFDPRVWVREGEKTMGAKITKSLETFRTTNTL

SEQ ID NO: 113 - protein, 358 aa, synthetic construct
MGILDIVPTGVITGDNVLKLFTYAREHGFAIPAINVTSSSTAIAALEAAREARSPIILQTSNGGAHFFAGKESSNEGQKASIAGSIAAAHYIRSIAPFFGVPVVMHSDHCAKKLLPWMDGMFEADEAYFKIHGEPLFSSHMLDLSEEPKKENIAQVKEYCKRAVPMKIWIEMEIGITGGEEDGVDNSHVSHTELYTQPEDIWDVYRELSSVTPYFSIAAAFGNVHGVYKPGNVKLQPALLGQHQAYVKEQLKTTNDKPVFFVFHGGSGSSVNEFRTGIKCGVVKVNIDTDTQFAYVEGVRDYVLKYKDYLMTPVGNPEGADKPNKKKFDPRVWIHEGEKTMTKRVLTALEDFYTVNTL

SEQ ID NO: 114 - protein, 363 aa, synthetic construct
MPHSYPALSAEQKKELSDIALRIVAPGKGILAADESVGSMAKRLSQIGVENTEENRRLYRQVLFSADDRVKKCIGGVIFFHETLYQKDDNGVPFVRTIQEKGILVGIKVDKGVVPLAGTDGETTTQGLDGLLERCAQYKKDGADFAKWRCVLKISDRTPSALAILENANVLARYASICQQNGIVPIVEPEILPDGDHDLKRCQFVTEKVLAAVYKALSDHHVYLEGTLLKPNMVTPGHACPIKYSPEEIAMATVTALRRTVPPAVPGVTFLSGGQSEEEASLNLNAINRCSLPRPWALTFSYGRALQASALSAWRGQRDNAGAATEEFIKRAEMNGLAAQGKYEGSGDGGAAAQSLYVANHAY

SEQ ID NO: 115 - protein, 364 aa, synthetic construct
MTHQFPALSPEQKKALSDIAQRIVASGKGILAADESVGTMGNRLQRINVENTEENRRAFREILFSSDASISKSIGGVILFHETLYQKDSSGKPFPAIIKEKGMVVGIKLDAGTAPLAGTNGETTIQGLDKLAERCAQYKKDGADFGKWRAVLKISSTTPSQLAIQENANTLARYASICQQNGLVPIVEPEVLPDGDHDLQRCQYVTEKVLAAVYKALNDHHVYLEGTLLKPNMVTAGHSCPKKYTPQDVAVATVTTLLRTVPAAVPGICFLSGGQSEEEASLNLNAMNQSPLPKPWKLTFSYGRALQASALAAWLGKSENKKAAQEAFCKRAQINSLACRGQYVTSGKTDTAATQSLFTASYTY

SEQ ID NO: 116 - protein, 391 aa, synthetic construct
MSAAADRLNLTSGHLNAGRKRSSSSVSLKAAEKPFKVTVIGSGNWGTTIAKVVAENCKGYPEVFAPIVQMWVFEEEINGEKLTEIINTRHQNVKYLPGITLPDNLVANPDLIDSVKDVDIIVFNIPHQFLPRICSQLKGHVDSHVRAISCLKGFEVGAKGVQLLSSYITEELGIQCGALSGANIATEVAQEHWSETTVAYHIPKDFRGEGKDVDHKVLKALFHRPYFHVSVIEDVAGISICGALKNVVALGCGFVEGLGWGNNASAAIQRVGLGEIIRFGQMFFPESREETYYQESAGVADLITTCAGGRNVKVARLMATSGKDAWECEKELLNGQSAQGLITCKEVHEWLETCGSVEDFPLFEAVYQIVYNNYPMKNLPDMIEELDLHED

SEQ ID NO: 117 - protein, 385 aa, synthetic construct
MSGYGQQGVSAANIDSIRPKKRLSIGVVGSGNWGTAIAKICGENARAHGHHFRSKVRMWVFEEEIEYKGEKRKLTEVFNEAHENVKYLPGIECPPNVIAVPDVREVARRADILVFVVPHQFIERVCDQMVGLIRPGAVGISCIKGVAVSKEGVRLYSEVISEKLGIYCGVLSGANVANEVAREQFCETTIGFNPPNEVDIPREQIAAVFDRPYFSVVSVDDVAGVALGGALKNVVAMAVGFADGLEWGGNTKAAIMRRGLLEMQKFATTFFDSDPRTMVEQSCGIADLVTSCLGGRNNRCAEAFVKTGKSLETLEKELLGGQLLQGAATSKDVHEFLLTKDMVKDFPLFTAVYNISYEDMDPKDLIIVLQPLKEDSENEGGTETE

SEQ ID NO: 118 - protein, 268 aa, synthetic construct
MTFTKWYWRVTVTASLGEETAFLCEVQQGGIFSIAGIEGTQMAHCLGAYCPNILFPYARECITSMVSRGTFPQLNLAPVNFDALFMNYLQQQAGEGTEEHQDALMNQRNASMTVIGAGSYGTALAITLARNGHEVVLWGHDPEHIATLERDRCNAAFLPDVPFPDTLHLESDLATALAASRNILVVVPSHVFGEVLRQIKPLMRPDARLVWATKGLEAETGRLLQDVAREALGDQIPLAVISGPTFAKELAAVTDGHFAGLYRPDLCR

SEQ ID NO: 119 - protein, 182 aa, synthetic construct
MQLGGAVKNVIAIGAGMSDGIGFGANARTALITRGLTEMSRLGAALGADPATFMGMAGLGDLVLTCTDNQSRNRRFGMMLGQGMDVKGAQDKIGQVVEGYRNTKEVRELAHRFGVEMPITEEIYQVLYCGKNAREASINVIRSRPQGRAESPLAVRNCLHKRPNPHRTGWSFSARLGVSHAV

SEQ ID NO: 120 - protein, 349 aa, synthetic construct
MAGKKVCIVGSGNWGSAIAKIVGSNAGRLAHFDPRVTMWVFEEDIGGRKLTEIINTQHENVKYLPGHKLPPNVVAIPDVVQAATGADILVFVVPHQFIGKICDQLKGHLKANTIGISLIKGVDEGPNGLKLISEVIGERLGIPMSVLMGANIASEVAEEKFCETTIGCKDPAQGQLLKDLMQTPNFRITVVQEVDTVEICGALKNIVAVGAGFCDGLGFGDNTKAAVIRLGLMEMIAFAKLFCSGTVSSATFLESCGVADLITTCYGGRNRKVAEAFARTGKSIEQLEKEMLNGQKLQGPQTARELHSILQHKGLVDKFPLFTAVYKVCYEGQPVGEFIRCLQNHPEHM

SEQ ID NO: 121 - protein, 351 aa, synthetic construct
MAAPLKVCIVGSGNWGSAIARIIGSNAQKLQCFATTVKMWVYEEMVNGKKLSEIINTEHENVKYLPGYKLPENVVAVPQLRDAADGADLLVFVVPHQFIRKLCDEMMGCVSERARGITLIKGIDEGPEGLKLISDIIREKMGIDVSVLMGANIANEVAAEKFCESTIGSKVLENGLLFKDLLQTPNFRITVVDDADTVELCGALKNIVAVGAGFCDGLQCGDNTKAAVIRLGLMEMIAFAKLFSKDDSVSSATFLESCGVADLITTCYGGRNRRVAEAFAKTGKSIEELEKEMLNGQKLQGPLTSAEVYHILKQKGLVEKFPLFTAVYQICFEDKPVRDMITCLQSHPEHL

SEQ ID NO: 122 - protein, 339 aa, synthetic construct
MNQRNASMTVIGAGSYGTALAITLARNGHEVVLWGHDPEHIATLERDRCNAAFLPDVPFPDTLHLESDLATALAASRNILVVVPSHVFGEVLRQIKPLMRPDARLVWATKGLEAETGRLLQDVAREALGDQIPLAVISGPTFAKELAAGLPTAISLASTDQTFADDLQQLLHCGKSFRVYSNPDFIGVQLGGAVKNVIAIGAGMSDGIGFGANARTALITRGLAEMSRLGAALGADPATFMGMAGLGDLVLTCTDNQSRNRRFGMMLGQGMDVQSAQEKIGQVVEGYRNTKEVRELAHRFGVEMPITEEIYQVLYCGKNAREAALTLLGRARKDERSSH

SEQ ID NO: 123 - protein, 345 aa, synthetic construct
MKKVTMLGAGSWGTALALVLTDNGNEVCVWAHRADLIHQINELHENKDYLPNVKLSTSIKGTTDMKEAVSDADVIIVAVPTKAIREVLRQAVPFITKKAVFVHVSKGIEPDSLLRISEIMEIELPSDVRKDIVVLSGPSHAEEVGLRHPTTVTASSKSMRAAEEVQDLFINHNFRVYTNPDIIGVEIGGALKNIIALAAGITDGLGYGDNAKAALITRGLAEIARLGTKMGGNPLTFSGLTGVGDLIVTCTSVHSRNWRAGNLLGKGYKLEDVLEEMGMVVEGVRTTKAAYQLSKKYDVKMPITEALHQVLFNGQKVETAVESLMARGKTHEMEDLVNTFENQVK

SEQ ID NO: 124 - protein, 329 aa, synthetic construct
MKISILGAGAWGTALALQISRRHQVSLWTRNQAHIVDMQVTRANLQYLGDFAFGDQLAVEGDLGRALDGADLIVSVVPTNGFRNALKEIKRLGCDAPVVWASKGLEAATAKLPHEVAQDELGDSRHWGVLSGPSFAAELVRGLPTAVTLAANDAEFAARAGAMLHGGNFRVYTSTDVIGVSVGGALKNVLAIAAGISDGMQCGNNARAALITRGIAEMTRFGVALGGAKETFMGLTGAGDLILTCTGQYSRNREVGLRLANGQTLQEILKTLGHVAEGVHTAREVVKRAGQLGVEMPITQEVDQVLSHGRSPRQAMENLLSREQKSEAL

SEQ ID NO: 125 - protein, 361 aa, synthetic construct
MKIPRVYSLGLTDVNKFLVYNLAKYPEQPKIPDIVLLLKSDEQLSRFVSNDSKVSVTDYTNLRASTKFTQLMAAYQPPRFANGDHAPIENLTISSSSFQLKTELKKFQKSINQNSNILLLNPSMSATQTINQLYGNSPKKPNIYQCLSTHSLWGAGEFGVNNIGRGNLTITKVPKNSNAPISEQNNLIDMKNEPPFIQLLSKLREVDPVFVSYFNFQLLQMESLVIKACIEPLTDVFDCYNGDLLKMDKISEISGDLIDESCQILKIAHPELVDSPLGSIALNSERLLDVVFNNLNLNKEGGREIAKLQKRSKKQEIFETNGYLSSLAKKHKIKAPLNTTYSDILRAKYSLANNRGLNGRL

SEQ ID NO: 126 - protein, 336 aa, synthetic construct
MKSLAQQYDCLLIDLDGTVFRGRRATEGAVQSLAEVSSRKLFITNNASRSADEVAAHLRELGFDAAGSDVVTSAQSAARVLADQLPAGSPVLIVGTDALGAEVAAVGLRPVRRWDDGPVAVVQGLSMTTGWPELAEAALAIRAGALWVAANVDPTLPTERGLLPGNGSLVAALRTATGAEPQVAGKPGPQLMADAVARGDCRAPLVIGDRLDTDIEGAHAAGLPSLMVLSGVNSARDAVFAPPRQRPTYLGHDLRCLHHDGELLAIGSQPGWRVDVADATVTVSATGDQDGDDLSVVRAVASAIWDAHPDGRPVSIGAGDEVARDALRRWSLERGD

SEQ ID NO: 127 - protein, 304 aa, synthetic construct
MSETIARAASSAPVPILGGLSAIAERYDLILCDVWGVLHDGTRAHMGAGEALIRFRTLPEDGRRRRVILVSNAPRPWAGVRTILDGYGVPREAYDAILTSGDLTRRLIAEHPGERIHHLGPERDATIFDGLDIRLVAAGEADRVVCTGLFDDTTETADDYRETLAGFRARNVPMICANPDLVVEREKKLIPCAGLIAQAYAEIGGAVTYAGKPYRPVYEAALAMAAELDGGSAPDVARVLAVGDALRTDIAGAAAYGIPNLLVARGIHAEELGVLAEHDTLGEVSEWLARQEVRPDAVIERLVW

SEQ ID NO: 128 - protein, 321 aa, synthetic construct
MAEAEAGGDEARCVRLSAERAKLLLAEVDTLLFDCDGVLWRGETAVPGAPETLRALRARGKRLGFITNNSSKTRTAYAEKLRRLGFGGPVGPEAGLEVFGTAYCSALYLRQRLAGVPDPKAYVLGSPALAAELEAVGVTSVGVGPDVLHGDGPSDWLAVPLEPDVRAVVVGFDPHFSYMKLTKAVRYLQQPDCLLVGTNMDNRLPLENGRFIAGTGCLVRAVEMAAQRQADIIGKPSRFIFDCVSQEYGINPERTVMVGDRLDTDILLGSTCSLKTILTLTGVSSLEDVKSNQESDCMFKKKMVPDFYVDSIADLLPALQG

SEQ ID NO: 129 - protein, 321 aa, synthetic construct
MAEAEAGGDDGRCVRLNAERAQALLADVDTLLFDCDGVLWRGETAVPGAPETLTALRARGKRLAFITNNSSKTREAYAEKLRCLGFGAPAGPDAGREVFGTAYCTALYLRQRLTGPPAPKAYVLGSVALAAELEAVGVSCVGVGPEPLLGDGPGAWLDAPLEPDVRAVVVGFDPHFSYMKLTKAVRYLQQPDCLLVGTNMDNRLPLENGRFIAGTGCLVRAVEMAAQRQADIIGKPSRFIFDCVSQEYGIHPERTVMVGDRLDTDILLGVTCGLKTILTLTGVSSLRDVKSNQESDCMAKKKMVPDFYVDSIADLLPALQG

SEQ ID NO: 130 - protein, 250 aa, synthetic construct
MPLTTKPLSLKINAALFDVDGTIIISQPAIAAFWRDFGKDKPYFDAEHVIHISHGWRTYDAIAKFAPDFADEEYVNKLEGEIPEKYGEHSIEVPGAVKLCNALNALPKEKWAVATSGTRDMAKKWFDILKIKRPEYFITANDVKQGKPHPEPYLKGRNGLGFPINEQDPSKSKVVVFEDAPAGIAAGKAAGCKIVGIATTFDLDFLKEKGCDIIVKNHESIRVGEYNAETDEVELIFDDYLYAKDDLLKW

SEQ ID NO: 131 - protein, 250 aa, synthetic construct
MGLTTKPLSLKVNAALFDVDGTIIISQPAIAAFWRDFGKDKPYFDAEHVIQVSHGWRTFDAIAKFAPDFANEEYVNKLEAEIPVKYGEKSIEVPGAVKLCNALNALPKEKWAVATSGTRDMAQKWFEHLGIRRPKYFITANDVKQGKPHPEPYLKGRNGLGYPINEQDPSKSKVVVFEDAPAGIAAGKAAGCKIIGIATTFDLDFLKEKGCDIIVKNHESIRVGGYNAETDEVEFIFDDYLYAKDDLLKW

SEQ ID NO: 132 - protein, 275 aa, synthetic construct
MTVNISYLTDMDGVLIKEGEMIPGADRFLQSLTDNNVEFMVLTNNSIFTPRDLSARLKTSGLDIPPERIWTSATATAHFLKSQVKEGTAYVVGESGLTTALHTAGWILTDANPEFVVLGETRTYSFEAITTAINLILGGARFICTNPDVTGPSPSGILPATGSVAALITAATGAEPYYIGKPNPVMMRSALNTIGAHSEHTVMIGDRMDTDVKSGLEAGLSTVLVRSGISDDAEIRRYPFRPTHVINSIADLADCWDDPFGDGAFHVPDEQQFTD

SEQ ID NO: 133 - protein, 365 aa, synthetic construct
MLKVIQSPAKYLQGPDASTLFGQYAKNLADSFFVIADDFVMKLAGEKVLNGLHSHDISCHAERFNGECSHIEINRLIAILKQHGCRGVVGIGGGKTLDTAKAIGYYQKLPVVVIPTIASTDAPTSALSVIYTEAGEFEEYLIYPKNPDMVVMDTAIIAKAPVRLLVAGMGDALSTWFEAKACYDARATSMAGGQSTVAALSLARLCYDTLLAEGEKARFAAQAGVVTDALERIVEANTYLSGIGFESSGLAGAHAIHNGFTILEECHHLYHGEKVAFGTLAQLVLQNSPMEEIETVLNFCQKVGLPVTLAEMGVKDDIDGKIMAVAKATCAEGETIHNMPFSVTPESVHAAILTADLLGQQWLAR

SEQ ID NO: 134 - protein, 275 aa, synthetic construct; identical to SEQ ID NO: 132

SEQ ID NO: 135 - protein, 99 aa, synthetic construct
IPGVGFGTFANEGATGXTYLKVDYIDLFLVHWPIAAEKAIGVSNWTIEGLEKENILPEAYSPLGIESNFKXGGYTLAQVLIAXGLSIQLTDXXYXAVNK

SEQ ID NO: 136 - protein, 331 aa, synthetic construct
MSSGKTVTLNSGYKIPQLGYGTWQAAPGEVGNGVYEALKIGYRHLDLAKIYENQKEVAEGIKRAYKDVPSLRREDIFITGKLWNTQHDPAIVEAALDDTLAELELEYLDLYLIHWPVNFGPGKNAHSDLFPMTSDPNEVNIDNSIPNSETWKAMTKLPKSKVRSVGVSNMTYQTLKGLVEKTGLVPAVNQIERHPILPSKELVAYAKEKNIHLTAYSAFGNNFFDIPLLIQRPEIKAIAEKKGATPAQVILAWSQVGGHSVIPKSVTPSRIAENFKEIDLDNEDIKAITKFSDEHQGRRRYNVPYTANKPRWSINIFNEPEEQKAPNSVVL

SEQ ID NO: 137 - protein, 283 aa, synthetic construct
MNNLTDTYTLNNGVKIPVVGFGTWQSKDGDEAYNAVKAALEAGYRHIDTAAAYGNEESVGKAIKDSGIDRKELFITSKLWNRDHGYESAKKALDTSLAKLGTDYLDLYLIHWPNPVQFRDEWQQRNADSWRAMEEALDAGKVRAIGVSNFRAHHLDELLKTAKVTPAVNQIFLNPSDTEDEVVAYNKEHGILSEAYSPLGTGKIFTIPELKDIAAKYNKSVAQVVLRWSLQHGFLPLPKSVHADRIKQNTEIFDFELSDDDIKKIDGFHGVAGLAQDPDTTDF

SEQ ID NO: 138 - protein, 286 aa, synthetic construct
MTALTKLTDTYTLNNGTKIPIVGFGTWQTPDGQVAYDSVLAALKAGYRHIDTAAAYGNEESVGKAIADSGVAREDLFVTTKLWNADHGYDAAKKALDTSLAKLGLDYVDLYLIHWPNPAAMRDNWEQLNADTWRAMEEAYTARKARAIGVSNFRPKHLDALLKTAKVVPAVNQIFLNPSDMEDEVVAYNRKHDILSEAYSPLGTGKIFSIPELKTLADKYDKSVAQVVLRWSLQHGFLPLPKSVHADRIKQNTELFDFELSDDDMKVIDGFHGVAGLANDPDQVNF

SEQ ID NO: 139 - protein, 312 aa, synthetic construct
MPATLHDSTKILSLNTGAQIPQIGLGTWQSKENDAYKAVLTALKDGYRHIDTAAIYRNEDQVGQAIKDSGVPREEIFVTTKLWCTQHHEPEVALDQSLKRLGLDYVDLYLMHWPARLDPAYIKNEDILSVPTKKDGSRAVDITNWNFIKTWELMQELPKTGKTKAVGVSNFSINNLKDLLASQGNKLTPAANQVEIHPLLPQDELINFCKSKGIVVEAYSPLGSTDAPLLKEPVILEIAKKNNVQPGHVVISWHVQRGYVVLPKSVNPDRIKTNRKIFTLSTEDFEAINNISKEKGEKRVVHPNWSPFEVFK

SEQ ID NO: 140 - protein, 316 aa, synthetic construct
MTVPEVCTKSYTLNTGASIPAIGLGTWRSTDDECYTAVMTALQNGYTHIDTARVYGNEEAVGRAINDFLKESKTPRERLFITTKLWCSECQNPEKALKKSLQRLNLDYVDLYLTHWPVAIDPNSSELMPTNESGQRMVLPFEEWSYLDTYRGMQKLVTLGLTKAIGISNYNIPKIKRLLADPEIKIVPACLQVEMHPCLPQNDLVEFCKSNNIVVQCYSPLGSTGAPVLQDETLKKIAASKNVHPATVAISWAVARDTVVLPKSVNPERIISNLKVIELSDDCVKEISEIGERNPKRVVNPEWTVKKNIFENFDYY

SEQ ID NO: 141 - protein, 152 aa, synthetic construct [sequence omitted]

SEQ ID NO: 142 - protein, 137 aa, synthetic construct
MKIALIAHDKKKQDMVQFTTAYRDILKNHDLYATGTTGLKIHEATGLQIERFQSGPLGGDQQIGALIAANALDLVIFLRDPLTAQPHEPDVSALIRLCDVYSIPLATNMGTAEILVRTLDEGVFEFRDLLRGEEPNV

SEQ ID NO: 143 - protein, 155 aa, synthetic construct
MDKKKRIALIAHDRRKRDLLEWVSFNLGTLSKHELYATGTTGALLQEKLGLKVHRLKSGPLGGDQQIGAMIAEGKIDVLIFFWDPLEPQAHDVDVKALIRIATVYNIPVAITRSTADFLISSPLMNDVYEKIQIDYEEELERRIRKVVEGEEEET

SEQ ID NO: 144 - protein, 249 aa, synthetic construct; identical to SEQ ID NO: 96

SEQ ID NO: 145 - protein, 249 aa, synthetic construct
MAPSRKFFVGGNWKMNGRKQSLGELIGTLNAAKVPADTKVVCAPPTAYIDFARQKLDPKIAVAAQNCYKVTNGAFTGEISPGMIKDCGATWVVLGHSERRHVFGESDELIGQKVAHALAEGLGVIACIGEKLDEREAGITEKVVFEQTKVITDNVKDWSKVVLAYEPVWAIGTGKTATPQQAQEVHEKLRGWLKSNVSDAVAQSTRIIYGGSVTGATCKELASQPDVDGFLVGGASLKPEFVDIINAKQ

SEQ ID NO: 146 - protein, 248 aa, synthetic construct; identical to SEQ ID NO: 97

SEQ ID NO: 147 - protein, 350 aa, synthetic construct
MSEQIPKTQKAVVFDTNGGQLVYKDYPVPTPKPNELLIHVKYSGVCHTDLHARKGDWPLATKLPLVGGHEGAGVVVGMGENVKGWKIGDFAGIKWLNGSCMSCEFCQQGAEPNCGEADLSGYTHDGSFEQYATADAVQAAKIPAGTDLANVAPILCAGVTVYKALKTADLAAGQWVAISGAGGGLGSLAVQYARAMGLRVVAIDGGDEKGEFVKSLGAEAYVDFTKDKDIVEAVKKATDGGPHGAINVSVSEKAIDQSVEYVRPLGKVVLVGLPAHAKVTAPVFDAVVKSIEIKGSYVGNRKDTAEAIDFFSRGLIKCPIKIVGLSDLPEVFKLMEEGKILGRYVLDTSK

SEQ ID NO: 148 - protein, 347 aa, synthetic construct
MRAAVYQGPGEIAVEEVPKPDIESPDDAVIRVTHTAVCGSDLWFYRGDSDREAGSRVGHEPMGIVEEVGDDVTSVAPGDRVIAPFAISCGECEFCRQGLYTSCVEDESWGSEANGGGQGEYVKCPFADGTLVRVPDRYADDEDVLESLLPLTDVMGTGHHAAVSAGVGEGDTVVVVGDGAVGLCGVLAAQRLGAERIIAMGHHEDRLELATEFGATDTISARGDDAIERARDLTHGGANHVMECVGAASAMDSAIAIARPGGTVGYVGVPYGVEDGGLDVFTMFSDNITIRGGVAPVRAYAEELMADVLQGTLDPSPIFTKTVDLDGVPEGYAAMDDREAIKVLVKA

SEQ ID NO: 149 - protein, 339 aa, synthetic construct
MSMIKSYAAKEAGGELEVYEYDPGELRPQDVEVQVDYCGICHSDLSMIDNEWGFSQYPLVAGHEVIGRVVALGSAAQDKGLQVGQRVGIGWTARSCGHCDACISGNQINCEQGAVPTIMNRGGFAEKLRADWQWVIPLPENIDIESAGPLLCGGITVFKPLLMHHITATSRVGVIGIGGLGHIAIKLLHAMGCEVTAFSSNPAKEQEVLAMGADKVVNSRDPQALKALAGQFDLIINTVNVSLDWQPYFEALTYGGNFHTVGAVLTPLSVPAFTLIAGDRSVSGSATGTPYELRKLMRFAARSKVAPTTELFPMSKINDAIQHVRDGKARYRVVLKADF

SEQ ID NO: 150 - protein, 399 aa, synthetic construct
MWETKINPNKVFELRCKNTTYFGIGSIKKIKDILEVLKNKGINNVILVTGKGSYKASGAWDVVKPALETLGFKYSLYDKVGPNPTVDMIDEAAKIGRETGAKAVIGIGGGSPIDTAKSVAVLLEYTDKNARELYEQKFIPEKAAPIIAINLTHGTGTEVDRFAVATIPEKNYKPAIAYDCLYPMYAIDDPSLMTKLDKKQTIAVTIDALNHVTEAATTLVASPYSVLMAKETVRLIVRYLPAAVNDPENLVARYYLLYASALAGISFDNGLLHLTHALEHPLSAVKPEIAHGLGLGAILPAVVKAIYPSVAEVLAEVYSPIVPGLKGLPAEAEYVAKKVEEWLFKVGCTQKLSDFGFTKEDIPTLVRLAKTTPSLDGLLSNAPVEATEAVIAKIYEESF

SEQ ID NO: 151 - protein, 312 aa, synthetic construct
MANKIFKLNTGAEIPALAFGTWQGEGDKVKAAVSYALQNGYKAVDCAYCYANEDAVGEGLREAFASGVKRSDIFITTKVWCTYQTSPERVEEGVDKSLKSLGLDYLDLVMIHWPVAMNPEGNHDRFPTLPDGKRDIIHGHSHIDTWKSLEKLLATGKAKAIGVSNYSKRYLEQLLPHVTVTPAVNQIENHPSLPQQEIVDFCKEKGIHIMAYSPFGSTGSPMFKAEPVVKVAEKKGVSPGTILLSYNVARGSTVIAKSVTPERILQNLQIVDLDEEDLKTLNDYSDELAKKGELKRYVYPPFGIDFGFPDKS

SEQ ID NO: 152 - protein, 324 aa, synthetic construct
MPIPTHFTLNTDAQIPAVGFGTWQAKPGEVERAVETALKAGYRHIDCAAIYRNEAEVGDGIRRSGVPRSEIFLTGKLWNTKHAPEDVESALDKSLQDLGVEYLDLFLMHWPVAFNGKPGKWFPLRESGVFDLADIDPATTYKAMEKLLSTGKVRAIGVSNFTINRLTDLLSKTNIVPAVNQIEAHPYLQQPALFDFCKSKGILIEAYSPLGNNQTGEPRTVDDELVGVLGRRLSLDGGQLLASWGIQRGTVVLPKSVTPSRIKSNMQVKELSKDTFEELNGLEKHKRFNVQSRWGFDIFEELGDEQVQKIAEDFAEENKTKFTV

SEQ ID NO: 153 - protein, 325 aa, synthetic construct
MTASSVLLHTGQKMPLIGLGTWKSEPGQVKAAIKHALSAGYRHIDCASVYGNETEIGEALKESVGSGKAVPREELFVTSKLWNTKHHPEDVEPALRKTLADLQLEYLDLYLMHWPYAFERGDNPFPKNADGTVRYDSTHYKETWKALEVLVAKGLVKALGLSNFNSRQIDDVLSVASVRPAVLQVECHPYLAQNELIAHCHARGLEVTAYSPLGSSDRAWRHPDEPVLLEEPVVLALAEKHGRSPAQILLRWQVQRKVICIPKSINPSRILQNIQVFDFTFSPEEMKQLDALNKNWRYIVPMITVDGKRVPRDAGHPLYPFNDPY

SEQ ID NO: 154 - protein, 277 aa, synthetic construct
MSSDRPVALVTGANKGIGFAIVRDLCRKFLGDVVLTARDESRGHEAVKQLQTEGLSPRFHQLDIDNPQSIRALRDFLLQEYGGLNVLVNNAGIAFKVVDPTPFHIQAEVTMKTNFFGTQDVCKELLPIIKPQGRVVNVSSSVSLRALKSCSPELQQKFRSETITEEELVGLMNKFIEDAKKGVHAKEGWPNSAYGVTKIGVTVLSRIYARKLNEERREDKILLNACCPGWVRTDMAGPKATKSPEEGAETPVYLALLPPGAEGPHGQFVQDKKVEPW

SEQ ID NO: 155 - protein, 277 aa, synthetic construct
MSSSNCVALVTGANKGIGFVIVRDLCRRFSGDVVLTARDEARGRAAVQQLQAEGLSPLFHQLDIDDRQSIRALRDFLRKEYGGLDVLVNNAGIAFKTADTTPFHIQAEVTMKTNFFGTRDVCTELLPLIKPQGRVVNVSSFVSVNSLKKCSRELQQKFRSETITEEELVGLMNKFVEDTKNGVHRKEGWPDTAYGVTKIGVTVLSRIHARKLSEQRGGDKILLNACCPGWVRTDMGGPKASKSPEEGAETPVYLALLPSDAEGPHGEFISEKRVVQW

SEQ ID NO: 156 - protein, 289 aa, synthetic construct
MSSNTRVALVTGANKGIGFAIVRDLCRQFAGDVVLTARDVARGQAAVKQLQAEGLSPRFHQLDIIDLQSIRALCDFLRKEYGGLDVLVNNAAIAFQLDNPTPFHIQAELTMKTNFMGTRNVCTELLPLIKPQGRVVNVSSTEGVRALNECSPELQQKFKSETITEEELVGLMNKFVEDTKNGVHRKEGWSDSTYGVTKIGVSVLSRIYARKLREQRAGDKILLNACCPGWVRTDMGGPKAPKSPEVGAETPVYLALLPSDAEGPHGQFVTDKKVVEWGVPPESYPWVNA

SEQ ID NO: 157 - protein, 351 aa, synthetic construct
MSSIPKEQWAQVIEKTGGPVEYKKIPVQQPGPDEVLVNIKYSGVCHTDLHAVNGDWPLETKLPLVGGHEGAGVVVARGDLVKDVEIGDYAGVKWLNGSCLACDYCQQADEPLCPKPLLSGYTVDGTFQQYCIAKAAHVARIPKECDLAAIAPVLCAGITVYKGLKESGVKPGQYAAIVGAGGGLGSLACQYAKAMGVRVVAIDTGDEKKKMCCGELGAETFVDFSTSKNLVADVQKATDGQGPHVVILVAVNEKPFQQAAEYVRPRGTVICIGLPAGAYLKAPVFDTVIKMVRIQGSYVGNRKDSSEAIEFFRRGLIKAPFKVVGLSELQMVYDKMHQGTIAGRYVLDTSK

SEQ ID NO: 158 - protein, 276 aa, synthetic construct
MPTSLKDTVKLHNGVEMPWFGLGVFKVENGNEATESVKAAIKNGYRSIDTAAIYKNEEGVGIGIKESGVAREELFITSKVWNEDQGYETTLAAFEKSLERLQLDYLDLYLIHWPGKDKYKDTWRALEKLYKDGKIRAIGVSNFQVHHLEELLKDAEIKPMVNQVEFHPRLTQKELRDYCKGQGIQLEAWSPLMQGQLLDNEVLTQIAEKHNKSVAQVILRWDLQHGVVTIPKSIKEHRIIENADIFDFELSQEDMDKIDALNKDERVGPNPDELLF

SEQ ID NO: 159 - protein, 281 aa, synthetic construct
MKNSKDYVILNNGVKMPLLGFGTYNAENLAKLKDSIKESIKIGYRHIDTASFYGNEEVIGGAIEESDVCRDEIFLVDKVWNSEQGYEKTLNAFKNSIKKLKTDYLDLYLIHWPQSLNKETWKALEKLYKDGYVRAIGVSNFTINHLKNLIENAEIMPSINQIEFHPRLVQKDLIEFCEKYDIQLEAWSPLMRGGVFQIPLLQEVAKKYQRTISQIVLRWDLQMGVATIPKSTTSARIKENSDIFNFEISKEDMIEIEKLNDGFRIGMNPNEVYERPEIIRE

SEQ ID NO: 160 - protein, 342 aa, synthetic construct
MSVFVSGANGFIAQHIVDLLLKEDYKVIGSARSQEKAENLTEAFGNNPKFSMEVVPDISKLDAFDHVFQKHGKDIKIVLHTASPFCFDITDSERDLLIPAVNGVKGILHSIKKYAADSVERVVLTSSYAAVFDMAKENDKSLTFNEESWNPATWESCQSDPVNAYCGSKKFAEKAAWEFLEENRDSVKFELTAVNPVYVFGPQMFDKDVKKHLNTSCELVNSLMHLSPEDKIPELFGGYIDVRDVAKAHLVAFQKRETIGQRLIVSEARFTMQDVLDILNEDFPVLKGNIPVGKPGSGATHNTLGATLDNKKSKKLLGFKFRNLKETIDDTASQILKFEGRI

SEQ ID NO: 161 - protein, 340 aa, synthetic construct
MSVLITGANGFIASHIVDTLLNSGYTVIGTARSESKFEPLLGEFKKKYPNGNLSYEVVSDITAEGAFDDLLKKHPEIKYVLHTASPFSFGHDKSFEEAYFKPAVEGTKNVLKSIKRYAPQVTNVVVTSSFAAIQRFTPNYVKYTNQDWNPMKLEECKNEIEAYCASKTHAEKAAWDFVKNEKPNFKLTTVNPPYVFGPQVFDSAVSKTLNTSNELINRVVKTPPTDELVSQPSGLGVDVRDVAKFHQLAFEKESAVGTRLFIVSGHFTGQTILNILNKHLPNEKLAVGAPEKDNATGLVGYGIENVLESVGGYEFISLEKSIVDAASQYLKKFGSFKQVE

SEQ ID NO: 162 - protein, 362 aa, synthetic construct
MSNSDIRVVPGPANYFSHPGSLERLSDFFNADQLSRAVWVYGERALAGAEPFLPAAFHLPEAKKIRFTGHCSERDVAGLVQASGDDRAVVIGVGGGALLDSAKVLARRLGVPLVAIPTIAATCAAWTPLSVWYSDAGQALNFELFDDANFLVLVEPRIILNAPAEYLLAGIGDTLAKWYEAVVLAPQPEALPLTVRLGINGAQAIRDVLLASSETALADQRRGDLTQAFRDVVEAIIAGGGMVGGLGERYTRVAAAHAVHNGLTVLPQTDKFLHGTKVAYGILVQSALLGQDDVLAQLVQAYQHFNLPTTLAALEVDINNRAELDRIIAHTLRPGESIHYLPVTLTPEVLRAAFEKVEYFSR

SEQ ID NO: 163 - protein, 365 aa, synthetic construct
MLKVIQSPAKYLQGPDAAVLFGQYAKNLAESFFVIADDFVMKLAGEKVVNGLQSHDIRCHAERFNGECSHAEINRLMAILQKQGCRGVVGIGGGKTLDTAKAIGYYQKLPVVVIPTIASTDAPTSALSVIYTEAGEFEEYLIYPKNPDMVVMDTAIIAKAPVRLLVSGMGDALSTWFEAKACYDARATSMAGGQSTEAALSLARLCYDTLLAEGEKACLAAQAGVVTEALERIIEANTYLSGIGFESSGLAAAHAIHNGFTILEECHHLYHGEKVAFGTLAQLVLQNSPMDEIETVLGFCQRVGLPVTLAQMGVKEGIDEKIAAVAKATCAEGETIHNMPFAVTPESVHAAILTADLLGQQWLAR

SEQ ID NO: 164 - protein, 450 aa, synthetic construct
MIGPRLCAATPRFPLVSLAHRNSKVFALASSNAVAQRWGKRFYAPIETETPHKVGVEFEESKDRIFTSPQKYVQGRHAFTRSYMYVKKWATKSAVVLADQNVWNICANKIVDSLSQNGMTVTKLVFGGEASLVELDKLRKQCPDDTQVIIGVGGGKTMDSAKYIAHSMNLPSIICPTTASSDAATSSLSVIYTPDGQFQKYSFYPLNPNLIFIDTDVIVRAPVRFLISGIGDALSTWVETESVIRSNSTSFAGGVASIAGRYIARACKDTLEKYALSAILSNTRGVCTEAFENVVEANTLMSGLGFENGGLAAAHAIHNGMTAIHGPVHRLMHGEKVAYGTLVQVVLEDWPLEDFNNLASFMAKCHLPITLEELGIPNVTDEELLMVGRATLRPDESIHNMSKKFNPSQIADAIKAVDSYSQKWQEQTGWTERFRLPPSRHSPHLTDIHP

SEQ ID NO: 165 - protein, 479 aa, synthetic construct
MSVPVQHPMYIDGQFVTWRGDAWIDVVNPATEAVISRIPDGQAEDARKAIDAAERAQPEWEALPAIERASWLRKISAGIRERASEISALIVEEGGKIQQLAEVEVAFTADYIDYMAEWARRYEGEIIQSDRPGENILLFKRALGVTTGILPWNFPFFLIARKMAPALLTGNTIVIKPSEFTPNNAIAFAKIVDEIGLPRGVFNLVLGRGETVGQELAGNPKVAMVSMTGSVSAGEKIMATAAKNITKVCLELGGKAPAIVMDDADLELAVKAIVDSRVINSGQVCNCAERVYVQKGIYDQFVNRLGEAMQAVQFGNPAERNDIAMGPLINAAALERVEQKVARAVEEGARVAFGGKAVEGKGYYYPPTLLLDVRQEMSIMHEETFGPVLPVVAFDTLEDAISMANDSDYGLTSSIYTQNLNVAMKAIKGLKFGETYINRENFEAMQGFHAGWRKSGIGGADGKHGLHEYLQTQVVYLQS

SEQ ID NO: 166 - protein, 382 aa, synthetic construct
MSFMLALPKISLHGAGAIGDMVNLVADKQWGKALIVTDGHLVEMGLLDSLFQALEAHQLSYHLFDNVFPNPTEALVQQGIAAFRAAQCDYIIAFGGGSPIDTAKAVKILSANPAPSTAYSGVGKVKNAGVPLVAINTTAGTAAEMTSNAVIIDSERQVKEVIIDPNIIPDIAVDDASVMLDIPPSVTAATGMDALTHAIEAFVSVGAHPLTDANALEAIRLIHQWLPLAVDDGHNLQAREQMAYGQYLAGMAFNSAGLGLVHALAHQPGATHNLPHGVCNAILLPIIENFNRPNAVARFARIAQAMGVDTRGMSDETASMAAINAIRALSKRVGIPEGFSQLGVSKADIEGWLDKALADPCAPCNPRSASRDEVRELYLEAL

SEQ ID NO: 167 - protein, 506 aa, synthetic construct
MSLDSLKGLGIKVPYKNKYDNYIGGQWVAPVDGEYFDNISPVTGKVFCQVPRSNEKDINLALDAAHAAKEAWARTSGTGRANILLKIADVMEANLETIAIAETIDNGKPIRETMAADIPLAIDHFRYFASCIRTQEGGISEIDHETVAYHFHEPLGVVGQIIPWNFPILMAAWKLAPALAAGNCIVMKPAEQTPASILVVMELIGDLLPPGVLNVVNGHGVEAGKALATSPRIAKIAFTGSTSVGRLIMQYASQNLIPVTLELGGKSPNIFFEDVMDKDDAYFDKALEGFTLFALNQGEICTCPSRALIQESIYEQFIERAIKRVKAIKQGSPLDKSTMIGAQASSEQVEIIMSYIKLGLEEGAQLLTGGNATKLPGDLSEGYYIEPTVFKGHNKMRIFQEEIFGPVLSVTTFKDEKEALEIANDTMYGLGAGLWTRDGSRAYRVGRGIQAGRVWTNCYHLYPAHAAFGGYKQSGIGRENHRMMLDHYQQTKNLLVSYSPNALGFF

SEQ ID NO: 168 - protein, 526 aa, synthetic construct
MSNDLKASLTFPEGHSVDKVEFPVGLFINNEYSPAANGETIEVRSPANDKVIAHVPAGQPEDVDRAVEAAQKAYDTVWGERCPGRERGRLLMKLADLFEEHVEQLASIEAMDNGKAFNIAKGFDVMEAAGCLRYYGGWADKDHGKMIEVDETKMAFERHEPIGVVGQIIPWNFPILMFAWKLGPALACGNTIVIKIAETTPLSAFYATQLIAKVFPPGVVNVVTGYGNVVGAAISSHMKILKVAFTGSTAVGRTIMQAAAKSNLKPVTLELGGKSPNIIFEDADLEQAVSWAAFGLYFNAGQCCCAGSRIFVQESIYDKFLELLTEKIKGMKVAQPFQPDAFVGPATSKLQFDRISAHIQSGKDEGATVHLGGERHGTEGYFLQPTVFTDVKPTMKIAQEEIFGPVVVVQTFRDDSDIIAKANDTFYGLAAAVFSRDISHALSTAKRLHAGTVWVNCYNQLNSSVPFGGFKQSGIGRELGEAALANCAPDFIMIVRGPRDADRRSSPLTDTAVKSIHVNLTQPNPL

SEQ ID NO: 169 - protein, 350 aa, synthetic construct
MSEQIPKTQKAVVFDTNGGQLVYKDYPVPTPKPNELLIHVKYSGVCHTDLHAWKGDWPLATKLPLVGGHEGAGVVVGMGENVKGWKIGDFAGIKWLNGSCMSCEFCQQGAEPNCGEADLSGYTHDGSFEQYATADAVQAAKIPAGTDLANVAPILCAGVTVYKALKTADLAAGQWVAISGAGGGLGSLAVQYARAMGLRVVAIDGGDEKGEFVKSLGAEAYVDFTKDKDIVEAVKKATDGGPHGAINVSVSEKAIDQSVEYVRPLGKVVLVGLPAHAKVTAPVFDAVVKSIEIKGSYVGNRKDTAEAIDFFSRGLIKCPIKIVGLSDLPEVFKLMEEGKILGRYVLDTSK

SEQ ID NO: 170 - protein, 191 aa, synthetic construct
MVKVCLFVADGTDEIEFSAPWGIFKRAEIPIDSVYVGENKDRLVKMSRDVEMYANRSYKEIPSADDFAKQYDIAIIPGGGLGAKTLSTTPFVQQVVKEFYKKPNKWIGMICAGTLTAKTSGLPNKQITGHPSVRGQLEEGGYKYLDQPVVLEENLITSQGPGTAMLFGLKLLEQVASKDKYNAVYKSLSMP

SEQ ID NO: 171 - protein, 236 aa, synthetic construct
MVKVLLALTSYNETFYSDGKKTGVFVVEALHPFEVFRKKGYEIQLASETGTFGWDDHSVVPDFLNGEDKEIFDNVNSEFNVALKNLKKASDLDPNDYDIFFGSAGHGTLFDYPNAKDLQKIATTVYDKGGVVSAVCHGPAIFENLNDPKTGEPLIKGKKITGFTDIGEDILGVTDIMKKGNLLTIKQVAEKEGATYIEPEGPWDNFTVTDGRIVTGVNPQSAVKTAEDVIAAFECN

SEQ ID NO: 172 - protein, 283 aa, synthetic construct [sequence omitted]

SEQ ID NO: 173 - protein, 229 aa, synthetic construct
MEQKKALIVVTSVEKYPNMERATGLWLGEAVHFYDKMVNAGKEVDFVSPRGGYTPLDPVSIQQFVQPVDWKYYADGTFRNKLADTLKPEEVNASDYDVIYYAGGHGVVWDFPEDKGLQNIARTIYENQGIISSVCHGAVGLFNITLSDGSLLIKDKTVTGFSNSEEIAAELADHMPYLTEDVLKSKGANYVKAEQDFTPFAVTDGRLVTGQNPQSGGAVGDQVLEILNQ

SEQ ID NO: 174 - protein, 135 aa, synthetic construct
MRLLHTMLRVGDLQRSIDFYTKVLGMKLLRTSENPEYKYSLAFVGYGPETEEAVIELTYNWGVDKYELGTAYGHIALSVDNAAEACEKIRQNGGNVTREAGPVKGGTTVIAFVEDPDGYKIELIEEKDAGRGLGN

SEQ ID NO: 175 - protein, 176 aa, synthetic construct
MSFNTEVQPGICMEPDAITQEYVFNHTMLRVKDPKRSLDFYSRVLGMRLLRRLDFEEGRFSLYFLAMTRGEEVPDAVDERQRYTFGRQSVLELTHNWGSESDDSQYHNGNQDPRGFGHICFSVPDLVAACERFETLGVNFVKPLDRGMKNVAFISDPDGYWVEIVQASLNGEMGRG

SEQ ID NO: 176 - protein, 131 aa, synthetic construct
MRILHTMLRVGDLDRSIKFYTEILGMQVLRREDYPDGKFTLAFVGYGGERDHTVLELTHNWGTESYDHGNAFGHIAIEVEDAYQACDKVKAAGGKVIREAGPMMHGTTVIAFIQDPDGYKIEFIQKGTAGY

SEQ ID NO: 177 - protein, 326 aa, synthetic construct
MSTDSTRYPIQIEKASNDPTLLLNHTCLRVKDPARTVKFYTEHFGMKLLSRKDFEEAKFSLYFLSFPKDDIPKNKNGEPDVFSAHGVLELTHNWGTEKNPDYKINNGNEEPHRGFGHICFSVSDINKTCEELESQGVKFKKRLSEGRQKDIAFALGPDGYWIELITYSREGQEYPKGSVGNKFNHTMIRIKNPTRSLEFYQNVLGMKLLRTSEHESAKFTLYFLGYGVPKTDSVFSCESVLELTHNWGTENDPNFHYHNGNSEPQGYGHICISCDDAGALCKEIEVKYGDKIQWSPKFNQGRMKNIAFLKDPDGYSIEVVPHGLIA

SEQ ID NO: 178 - protein, 302 aa, synthetic construct
MASTTDMSTYKLNHTMIRVKDLDKSLKFYTEVFGMKLIDQWVFEENEFSLSFLAFDGPGALNHGVERSKREGILELTYNFGTEKKEGPVYINGNTEPKRGFGHICFTVDNIESACAYLESKGVSFKKKLSDGKMKHIAFALDPDNYWIELVSQSETKPKANISNFRFNHTMVRVKDPEPSIAFYEKLGMKVIDKADHPNGKFTNYFLAYPSDLPRHDREGLLELTHNWGTEKESGPVYHNGNDGDEKGYGHVCISVDNINAACSKFEAEGLPFKKKLTDGRMKDIAFLLDPDNYWVEVIEQK

SEQ ID NO: 179 - protein, 184 aa, synthetic construct
MAEPQPASSGLTDETAFSCCSDPDPSTKDFLLQQTMLRIKDPKKSLDFYTRVLGLTLLQKLDFPAMKFSLYFLAYEDKNDIPKDKSEKTAWTFSRKATLELTHNWGTEDDETQSYHNGNSDPRGFGHIGIAVPDVYSACKRFEELGVKFVKKPDDGKMKGLAFIQDPDGYWIEILNPNKIATII

SEQ ID NO: 180 - protein, 251 aa, synthetic construct
MNLNSIPAFDDNYIWVLNDEAGRCLIVDPGDAEPVLNAIAANNWQPEAIFLTHHHHDHVGGVKELVEKFPQIVVYGPQETQDKGTTQVVKDGETAFVLGHEFSVIATPGHTLGHICYFSKPYLFCGDTLFSGGCGRLFEGTASQMYQSLKKLSALPDDTLVCCAHEYTLSNMKFALSILPHDLSINDYYRKVKELRAKNQITLPVILKNERQINVFLRTEDIDLINVINEETLLQQPEERFAWLRSKKDRF

SEQ ID NO: 181 - protein, 250 aa, synthetic construct
MFEIIPILAFEDNYIWLLHQHGHALVVDPGDAHPVLEILDARGLQLRAILVTHHHQDHTGGVEELIQATSAQVFAPAKEQFSFPHHPVTAGDRLDIPGIALSLSVLDVPGHTVGHVAYYGDGMLFSGDTLFGAGCGRLFEGTPGQMYSSLQQLAQLPVNTRVYCGHEYTERNLAFALSLEPHHEALLSRREATAALRAQGLPSLPSSMALELATNPFLRCHEPGIIAASKSAATDPVSVFAAIREMRNHF

SEQ ID NO: 182 - protein, 256 aa, synthetic construct
MSFHITPIWMWKGTGNNYAYLLTCDKTKITAIVDPAEPESVIPVIKEKTAKKEIDLQYILTTHHHYDHAGGNEDILSYFPSLKVYGGKNASGVTYTPKDKEIFKVGEVQVEALHTPCHTQDSICYYVSSPSKRAVFTGDTLFTSGCGRFFEGDAKQMDYALNHVLAALPDDTVTYPGHEYTKSNAKFSSTIFSTPELTKLVDFCKNHESTTGHFTIGDEKKFNPFMCLGLESVQKAVGSSDPITVMKKLRDMKNAA

SEQ ID NO: 183 - protein, 651 aa, synthetic construct
MAKVIFTPWKEHSQLLAVRSQFYPAPFYDGPDMRSKACATVAAWKLRGNLPHPVEATALLTDAILHDDALKNSIFSIRATYSAAFCRFVTGLVDSKLNGQRKTMFQRAIDLGLPASFVELRHEATHRELPSLTVLRNATQRSLEWLWDYYWAKTDLSADTVPVSEPEAFDGAEDDVEPIKAALRTEFEHLLAEEESSEPPRKKRRFQQNVSFTSTHLISICKSSSRGASALAGVIVEDSLLVPAGRKMGDSMTGMFAKWDSLLQMLAEGHPPALASLTEEMVNVLAFSGSKNAKSDPQLEGLYMWLDHILQSPEWGSRRRLLSHAYLLAVCEQSSNHWTALLKESLQQRTEDLAPKKPASTSKKQSKKDGSGLKRTADADDLKALKNFGWETVDTWDTRPFVLSGTGKGNNYAYLVTDEPTKESVIIDPANPPEVAPTLQSQIDAGKIKLTSIVNTHHHWDHAGGNNEILKTFGKLSVIGGKNCQSVTKTPAHGEVFKIGERISVKALHTPCHTQDSICYFMQDGDDKVVFTGDTLFIGGCGRFFEGTAPEMHKALNETLAALPDDTKVYPGHEYTKGNVKFCLAVSQSEPIKKLEAFANANQETQGKFTIGDEKLHNVFMRVNDPEIQKKTGKTDPVEVMAALREMKNSM

SEQ ID NO: 184 - protein, 309 aa, synthetic construct
MVLGRGSLCLRSLSVLGAACARRGLGQALLGLSLCHTDFRKNLTVQQDMMKIELLPALTDNYMYLIIDEDTQEAAVVDPVQPQKVIETVKKHRVKLTTVLTTHHHWDHAGGNEKLVKLEPGLKVYGGDDRIGALTHKVTHLSTLEVGSLSVKCLSTPCHTSGHICYFVSKPGSSEPSAVFTGDTLFVAGCGKFYEGTADEMYKALLEVLGRLPPDTKVICGHEYTVNNLKFARHVEPGNTAVQEKLAWAKEKNAIGEPTVPSTLAEEFTYNPFMRVKEKTVQQHAGETDPVTTMRAIRREKDQFKVPRD

SEQ ID NO: 185 - protein, 308 aa, synthetic construct
MVLGRGLLGRWSVAELGAVCARLGLGPALLGSLHHLGLRKSLTVDQGTMKVELLPALTDNYMYLLIDEDTKEAAIVDPVQPQKVVETARKHGVKLTTVLTTHHHWDHAGGNEKLVKLEPGLKVYGGDDRIGALTHKVTHLSTLQVGSLHVKCLSTPCHTSGHICYFVTKPNSPEPPAVFTGDTLFVAGCGKFYEGTADEMYKALLEVLGRLPADTRVYCGHEYTINNLKFARHVEPDNTAVREKLAWAKEKYSIGEPTVPSTIAEEFTYNPFMRVREKTVQQHAGETEPVATMRAIRKEKDQFKMPRD

SEQ ID NO: 186 - protein, 382 aa, synthetic construct
MANRMILNETAWFGRGAVGALTDEVKRRGYQKALIVTDKTLVQCGVVAKVTDKMDAAGLAWAIYDGVVPNPTITVVKEGLGVFQNSGADYLIAIGGGSPQDTCKAIGIISNNPEFADVRSLEGLSPTNKPSVPILAIPTTAGTAAEVTINYVITDEEKRRKFVCVDPHDIPQVAFIDADMMDGMPPALKAATGVDALTHAIEGYITRGAWALTDALHIKAIEIIAGALRGSVAGDKDAGEEMALGQYVAGMGFSNVGLGLVHGMAHPLGAFYNTPHGVANAILLPHVMRYNADFTGEKYRDIARVMGVKVEGMSLEEARNAAVEAVFALNRDVGIPPHLRDVGVRKEDIPALAQAALDDVCTGGNPREATLEDIVELYHTAW

SEQ ID NO: 187 - protein, 382 aa, synthetic construct; identical to SEQ ID NO: 166

SEQ ID NO: 188 - protein, 384 aa, synthetic construct
MINRFILNEVSYFGPGAREVLPKEISRLGLHKAFVATDKDLIKFGVADKVLKVLEAAKIPYEIFSEIKPNPTVSNVKAGVEAFASSGADFILAIGGGSSMDTAKAIGIITNNPEFSDVVSLEGVADTKKKSVPIIALPTTAGTAAEVTINYVITDEQNQKKMVCVDPNDIPSIAIVDAELMYTLPKSLTAATGLDALTHAIEGLITKGAWEMSDMFEIKAIEMINRYLVTAVEEPSNAEARNGMAVAQYIAGMAFSNVGLGVVHGMAHPLGAIFDIPHGVANALLLPIIMEFNAPAALDKYVEIAKAMNVYSTDMTKEKAAEAAVQAVKTLSLRVNIPQHLSDLGIQESDLDRLATAAFADVCTPGNPREVTKEIILDLYKKAL

SEQ ID NO: 189 - protein, 387 aa, synthetic construct
MEMGFFAPRHMDIGGGAAARIAVLLGRFGLSRPLIVTDPVMVKLGLVRRITDPLEAAGIVCTIFSDTVPEPVDTVVEAGVAIARGGAFDCLIGFGGGSPIDTAKAINILLAAAPSARMRDFKVPVAADTAALPLIAVPTTAGTGSEATRFTVITDTETDEKMLIAGLGALPLAAVVDYELTMSVPPRTTADTGIDAFTHALEAYVSRRANPVSDAYARSAMRLIGANLRKVWQTPQDRDAREAMMLGATLAGLAFSNASVALVHGMSRPIGAHFHVPHGMSNAMLLPAVTRFSLNAALPRYAESARLAGFARADDADQLAGARLIEALEAINAELEVPTPQGFGVARADWDALLPKMAEQALASGSPGNNPAVPDAAEIVKIYEEIF

SEQ ID NO: 190 - protein, 350 aa, synthetic construct
MIVEAYGAHAGEKPLEPMEIIRRAPGAHDVQIDIAYCGVCHSDIHQVRSEWPGTLYPCVPGHEIVGRVSAVGAHVVDFQVDDLVGIGCIVDSCQNCEECDVGLENYCDGMVGTYNGPTPDAPGHTLGGYSQQIVVHERYVLRIRHPEAQLAAVAPLLCAGITTYSPLRHWKTGPGKKVGIVGIGGLGHIGIKLAHAMGAHVVAFTTSESKREAAKALGADEAVVSRNADEMAAHAKSFDFILNTVAAPHDLDAFVVLLKRDGAMTLVGAPATPHPSPNVMNLILKRRSIAGSAIGGIPETQEMLDFCAERGIVSDIEMIRADEINEAYERMINGDVKYRFVIDNASLTAL

SEQ ID NO: 191 - protein, 406 aa, synthetic construct
MSNTNDKDRTNKMETAGHSRRGFMVSAATAVAGVSAANLLNLQTANAAITNNVVAIGNGPYPVEGMAAYSPAGPHRPMKFQRRTLGPKDVAIKIHYCGVCHSDIHTIRGDWGKIQYPQIVGHELAGEVVAVGSSASKFNVGARVGVGTMVNSCRVCTECQAGHESYCLNGNTQAYGSKDRDGTITQGGYSTFVVVDEDFVINIPAAIDLAEAGPLMCAGITVYSPLLRWGVSAGKKVAIVGMGGLGHLAVKIATALGAEVTVFTTSPDKVEDARRFGAKDVVINKEGADFSRFKHAFDFALDTVPYKHDLNRFIPLLKRDATYCRVGVGNVVDSNEIGQMNLVLYRNSLAGSNTGGIKETQDMIDFCALNKIKPEITKILMNGIDDAWTKVIEKKARYRYVMDMKA

SEQ ID NO: 192 - protein, 367 aa, synthetic construct
MDRIIQSPGKYIQGADVINRLGEYLKPLAERWLVVGDKFVLGFAQSTVEKSFKDAGLVVEIAPFGGECSQNEIDRLRGIAETAQCGAILGIGGGKTLDTAKALAHFMGVPVAIAPTIASTDAPCSALSVIYTDEGEFDRYLLLPNNPNMVIVDTKIVAGAPARLLAAGIGDALATWFEARACSRSGATTMAGGKCTQAALALAELCYNTLLEEGEKAMLAAEQHVVTPALERVIEANTYLSGVGFESGGLAAAHAVHNGLTAIPDAHHYYHGEKVAFGTLTQLVLENAPVEEIETVAALSHAVGLPITLAQLDIKEDVPAKMRIVAEAACAEGETIHNMPGGATPDQVYAALLVADQYGQRFLQEWE

SEQ ID NO: 193 - protein, 370 aa, synthetic construct
MAAERVFISPAKYVQGKNVITKIANYLEGIGNKTVVIADEIVWKIAGHTIVNELKKGNIAAEEVVFSGEASRNEVERIANIARKAEAAIVIGVGGGKTLDTAKAVADELDAYIVIVPTAASTDAPTSALSVIYSDDGVFESYRFYKKNPDLVLVDTKIIANAPPRLLASGIADALATWVEARSVIKSGGKTMAGGIPTIAAEAIAEKCEQTLFKYGKLAYESVKAKVVTPALEAVVEANTLLSGLGFESGGLAAAHAIHNGFTALEGEIHHLTHGEKVAFGTLVQLALEEHSQQEIERYIELYLSLDLPVTLEDIKLKDASREDILKVAKAATAEGETIHNAFNVTADDVADAIFAADQYAKAYKEKHRK

SEQ ID NO: 194 - protein, 555 aa, synthetic construct
MRRSKRFEVLAQRPVNQDGLIGEWPEEGLIAMESPYDPASSVKVENGRIVELDGKSRAEFDMIDRFIADYAINVPEAERAMQLDALEIARMLVDIHVSREEIIAITTAITPAKRLEVMAQMNVVEMMMALQKMRARRTPSNQCHVTNLKDNPVQIAADAAEAGIRGFSEQETTVGIARYAPFNALALLVGSQCGAPGVLTQCSVEEATELELGMRGLTSYAETVSVYGTESVFTDGDDTPWSKAFLASAYASRGLKMRYTSGTGSEALMGYSESKSMLYLESRCIFITKGAGVQGLQNGAVSCIGMTGAVPSGIRAVLAENLIASMLDLEVASANDQTFSHSDIRRTARTLMQMLPGTDFIFSGYSAVPNYDNMFAGSNFDAEDFDDYNILQRDLMVDGGLRPVTEEETIAIRNKAARAIQAVFRELGLPLISDEEVDAATYAHGSKDMPARNVVEDLAAVEEMMKRNITGLDIVGALSSSGFEDIASNILNMLRQRVTGDYLQTSAILDRQFDVVSAVNDINDYQGPGTGYRISAERWAEIKNIAGVVQPGSIE

SEQ ID NO: 195 - protein, 555 aa, synthetic construct
MKRSKRFAVLAQRPVNQDGLIGEWPEEGLIAMDSPFDPVSSVKVDNGLIVELDGKRRDQFDMIDRFIADYAINVERTEQAMRLEAVEIARMLVDIHVSREEIIAITTAITPAKAVEVMAQMNVVEMMMALQKMRARRTPSNQCHVTNLKDNPVQIAADAAEAGIRGFSEQETTVGIARYAPFNALALLVGSQCGRPGVLTQCSVEEATELELGMRGLTSYAETVSVYGTEAVFTDGDDTPWSKAFLASAYASRGLKMRYTSGTGSEALMGYSESKSMLYLESRCIFITKGAGVQGLQNGAVSCIGMTGAVPSGIRAVLAENLIASMLDLEVASANDQTFSHSDIRRTARTLMQMLPGTDFIFSGYSAVPNYDNMFAGSNFDAEDFDDYNILQRDLMVDGGLRPVTEAETIAIRQKAARAIQAVFRELGLPPIADEEVEAATYAHGSNEMPPRNVVEDLSAVEEMMKRNITGLDIVGALSRSGFEDIASNILNMLRQRVTGDYLQTSAILDRQFEVVSAVNDINDYQGPGTGYRISAERWAEIKNIPGVVQPDTIE

SEQ ID NO: 196 - protein, 554 aa, synthetic construct
MKSKRFEALAKRPVNQDGFVKEWIEEGFIAMESPNDPKPSIKIVNGVVTELDGKPQSSFDLIDHFIARYGINLAHAEKVMKMDSIKLANMLCDPNVSRRTIVPLTTAMTPAKIVEVVSHMNVVEMMMSMQKMRARRTPSQQAHVTNVKDNPVQIAADAAEGAFRGFDEQETTVAVARYAPFNAIALLVGSQVGRPGVLTQCSLEEATELKLGMLGHTCYAETISVYGTEPVFTDGDDTPWSKGFLASSYASRGLKMRFTSGSGSEVQMGYAEGKSMLYLEARCIYITKAAGVQGLQNGSVSCVGVPSAVPSGIRAILAENLICSALDLECASSNDQTFTHSDMRRTARLLMQFLPGTDFISSGYSAVPNYDNMFAGSNEDAEDFDDYNVLQRDLKVDGGLRPVLEADVVAIRNKAARALQAVFAGMGLPPITDEEVIAATYAHGSKDMPERNIVEDIKFAQEIINKNRTGLEVVKALAQGGFEDVAQDMLNIQKAKIAGDYLHTSAIIKGDNQVLSAVNDVNDYAGPATGYRLEGARWEEIKNIPNALDPNELG

SEQ ID NO: 197 - protein, 512 aa, synthetic construct
MTNNPPSAQIKPGEYGFPLKLKARYDNFIGGEWVAPADGEYYQNLTPVTGQLLCEVASSGKRDIDLALDAAHKVKDKWAHTSVQDRAAILFKIADRMEQNLELLATAETWDNGKPIRETSAADVPLAIDHFRYFASCIRAQEGGISEVDSETVAYHFHEPLGVVGQIIPWNFPLLMASWKMAPALAAGNCVVLKPARLTPLSVLLLMEIVGDLLPPGVVNVVNGAGGVIGEYLATSKRIAKVAFTGSTEVGQQIMQYATQNIIPVTLELGGKSPNIFFADVMDEEDAFFDKALEGFALFAFNQGEVCTCPSRALVQESIYERFMERAIRRVESIRSGNPLDSVTQMGAQVSHGQLETILNYIDIGKKEGADVLTGGRRKLLEGELKDGYYLEPTILFGQNNMRVFQEEIFGPVLAVTTFKTMEEALELANDTQYGLGAGVWSRNGNLAYKMGRGIQAGRVWTNCYHAYPAHAAFGGYKQSGIGRETHKMMLEHYQQTKCLLVSYSDKPLGLF

SEQ ID NO: 198 - protein, 534 aa, synthetic construct
MNASQTTAGRQFIAGRRVASGEATLLSLRAVDGEATGHRFYPASHAEAAQAAEAAQQAFAIYSQTAPQQRAHFLCAIADELDALGEAFFAIAEQETALPLARLQGERARTSGQLRMFAGVILRGDTFAARIDTALADRQPLPRPDLRQYQQALGPVAVFGASNFPLAFSTAGGDTASALAAGCPVVVKAHAGHMATAELTADAIVRAVARCGLPGGVFNMIFGTDIGAELVRHPAIQAVGFTGSLAGGKALYQLAQQRPQPIPLFAEMSAINPLIILPQALQTRAEALANALVASFTLGGGQFCTRPGLILALRGAGLERFKSALCAAVAGCAPQVLLNAPTLQHYRQGVAALAAHPRIERLASGLAAGAGQAQTQLWQAQVEDLLAQDALLQTEVFGPLSLLVEVDDAAQLQAVVKALQGQLTATLHAEADDGPLAASLLPLLCEKAGRVLFNGYPTGVEVCDAMVHGGPWPATTDARGTSVGSRAIERFLRPVCLQNAPAALLPPALQDANPLNLLRLVNGQWTREAISSSH

SEQ ID NO: 199 - protein, 366 aa, synthetic construct
MTAMMKAAVFVEPGRIELADKPIPDIGPNDALVRITTTTICGTDVHILKGEYPVAKGLTVGHEPVGIIEKLGSAVTGYREGQRVIAGAICPNFNSYAAQDGVASQDGSYLMASGQCGCHGYKATAGWRFGNMIDGTQAEYVLVPDAQANLTPIPDGLTDEQVLMCPDIMSTGFKGAENANIRIGDTVAVFAQGPIGLCATAGARLCGATTIIAIDGNDHRLEIARKMGADVVLNFRNCDVVDEVMKLTGGRGVDASIEALGTQATFEQSLRVLKPGGTLSSLGVYSSDLTIPLSAFAAGLGDHKINTALCPGGKERMRRLINVIESGRVDLGALVTHQYRLDDIVAAYDLFANQRDGVLKIAIKPH

SEQ ID NO: 200 - protein, 445 aa, synthetic construct
MEQQVKDDIQRVFQLQKKQQKALRASTAEQRREKLQRFLDSVIAHEEEIIEAIRKDVRKPYHEVKKAEIEGTKKAIRDNMNNLEQWMAPKEVGSSLSPDANGILMYEPKGVTLILGPWNYPFMLTMAPLAASLAAGNSAIVKLSDFTMNTSNIAAKVIRDAFDEKEVAIFEGEVEVATELLDQPFDHIFFTGSTNVGKIVMTAAAKHLASVTLELGGKSPTIIDSEYDLMDAAKKIAVGKFVNAGQTCIAPDYLFIKKDVQDRFAGILQTVVNAGFMEDDHTPDRSKFTQIVNDRNFNRVKDLFDDAIERGAEVVFGGVFDASDRTISPTVLKNVTPDMKIMQEEIFASILPMMNYEDIDEVIDYVNDRDKPLALYVFSKNQDLIDNVLQHTTSGNAAINDVVVHFSDVNLPFGGVNTSGIGSYHGVYGFKEFSHEKGVFIQAAE

SEQ ID NO: 201 - protein, 532 aa, synthetic construct
MSNDGSKILNYTPVSKIDEIVEISRNFFFEKQLKLSHENNPRKKDLEFRQLQLKKLYYAVKDHEEELIDAMYKDFHRNKIESVLNETTKLMNDILHLIEILPKLIKPRRVSDSSPPFMFGKTIVEKISRGSVLIIAPFNFPLLLAFAPLAAALAAGNTIVLKPSELTPHTAVVMENLLTTAGFPDGLIQVVQGAIDETTRLLDCGKFDLIFYTGSPRVGSIVAEKAAKSLTPCVLELGGKSPTFITENFKASNIKIALKRIFFGAFGNSGQICVSPDYLLVHKSIYPKVIKECESVLNEFYPSFDEQTDFTRMIHEPAYKKAVASINSTNGSKIVPSKISINSDTEDLCLVPPTIVYNIGWDDPLMKQENFAPVLPIIEYEDLDETINKIIEEHDTPLVQYIFSDSQTEINRILTRLRSGDCVVGDTVIHVGITDAPFGGIGTSGYGNYGGYYGFNTFSHERTIFKQPYWNDFTLFMRYPPNSAQKEKLVRFAMERKPWFDRNGNNKWGLRQYFSLSAAVILISTIYAHCSS

SEQ ID NO: 202 - protein, 461 aa, synthetic construct
MSFDTFYNIITGQPRSARETTSGVNPLDRSSLWPAPVATGNDVEEAVRSAQEAFPAWSEKTYKQRTELLEKFADLYLVHANEFCQLIATECGRTAGNAAIEVYVAAQWLRYPSKYEIPEEVTEDEKKTSIVTHEPLGVVAAICPWNFPLMLALGKIAPALATGNCVILKPSPFTPYSSLKLVELAQQVFPPSVLQVLHGHDDLGPMLVKHPRIQKITFTGSTTTGKQILRDAAETMKRVTLETAGNNASIILPDVNIEAVIPQLAGGLWFNAGQVCIATRRMYIHQDIFDEAVAQLAEASKDLASGMEPIQNEMQLVRLQQALSDANAAGCELLSLGKTEAAEGFFIQPTILKSPPPDADVVQQENFGPIVSCIKFSSLDEAISLANNSDTGLAASVWSSDVSAARRVAAKLEVGNVYINGPPQPDPYVPFGGHKQSGLGVEYGLPGLLSFCQTKSTYLYK

SEQ ID NO: 203 - protein, 501 aa, synthetic construct
MSSPAQPAVPAPLADLKIQHTKIFINNEWHNSVSGKKFPVLNPATEEVICHVEEGDKADVDKAVKAARQAFQIGSPWRTMDASERGRLLNKLADLMERDRLLLATMEALNGGKVFANAYLSDLGGCIKALKYCAGWADKIHGQTIPSDGDIFTYTRREPIGVCGQIIPWNFPMLMFIWKIGPALSCGNTVVVKPAEQTPLTALHLASLIKEAGFPPGVVNIVPGYGPTAGAAISSHMDVDKVAFTGSTQVGKLIKEAAGKSNLKRVTLELGGKSPCIVFADADLDIAVEFAHHGVFYHQGQCCVAASRIFVEESVYDEFVKRSVERAKKYVLGNPLTPGINQGPQIDKEQHDKILDLIESGKKEGAKLECGGGRWGNKGFFVQPTVFSNVTDEMRIAKEEIFGPVQQIMKFKSVDDVIKRANNTTYGLAAGLFTKDLDKAITVSSALQAGVVWVNCYMMLSAQCPFGGFKMSGNGRELGEHGLYEYTELKTVAMKISQKNS

SEQ ID NO: 204 - protein, 501 aa, synthetic construct
MSSSAMPDVPAPLTNLQFKYTKIFINNEWHSSVSGKKFPVFNPATEEKLCEVEEGDKEDVDKAVKAARQAFQIGSPWRTMDASERGRLLNKLADLIERDHLLLATMEAMNGGKLFSNAYLMDLGGCIKTLRYCAGWADKIQGRTIPMDGNFFTYTRSEPVGVCGQIIPWNFPLLMFLWKIGPALSCGNTVVVKPAEQTPLTALHMGSLIKEAGFPPGVVNIVPGYGPTAGAAISSHMDVDKVAFTGSTEVGKLIKEAAGKSNLKRVSLELGGKSPCIVFADADLDNAVEFAHQGVFYHQGQCCIAASRLFVEESIYDEFVRRSVERAKKYVLGNPLTPGVSQGPQIDKEQYEKILDLIESGKKEGAKLECGGGPWGNKGYFIQPTVFSDVTDDMRIAKEEIFGPVQQIMKFKSLDDVIKRANNTFYGLSAGIFTNDIDKAITVSSALQSGTVWVNCYSVVSAQCPFGGFKMSGNGRELGEYGFHEYTEVKTVTIKISQKNS

SEQ ID NO: 205 - protein, 224 aa, synthetic construct
MEINEKLLRQIIEDVLRDMKGSDKPVSFNAPAASTAPQTAAPAGDGFLTEVGEARQGTQQDEVIIAVGPAFGLAQTVNIVGLPHKSILREVIAGIEEEGIKARVIRCFKSSDVAFVAVEGNRLSGSGISIGIQSKGTTVIHQQGLPPLSNLELFPQAPLLTLETYRQIGKNAARYAKRESPQPVPTLNDQMARPKYQAKSAILHIKETKYVVTGKNPQELRVAL

SEQ ID NO: 206 - protein, 224 aa, synthetic construct
MEINEKLLRQIIEDVLSEMQTSDKPVSFRASTAASAPQAAAAQGDSFLTEIGEAKQGQQQDEVIIAVGPAFGLSQTVNIVGIPHKNILREVIAGIEEEGIKARVIRCFKSSDVAFVAVEGNRLSGSGISIGIQSKGTTVIHQQGLPPLSNLELFPQAPLLTLETYRQIGKNAARYAKRESPQPVPTLNDQMARPKYQAKSAILHIKETKYVVTGKNPQELRVAL

SEQ ID NO: 207 - protein, 554 aa, synthetic construct
MKSKRFEALAKRPVNQDGFVKEWIEEGFIAMESPNDPKPSIKIVNGVVTELDGKPQSSFDLIDHFIARYGINLDHAEEVMKMDSIKLANMLCDPNVSRRTIVPLTTAMTPAKIVEVVSHMNVVEMMMSMQKMRARRTPSQQAHVTNVKDNPVQIAADAAEGAFRGFDEQETTVAVARYAPFNAIALLVGSQVGRPGVLTQCSLEEATELKLGMLGHTCYAETISVYGTEPVFTDGDDTPWSKGFLASSYASRGLKMRFTSGSGSEVQMGYAEGKSMLYLEARCIYITKAAGVQGLQNGSVSCVGVPSAVPSGIRAILAENLICSALDLECASSNDQTFTHSDMRRTARLLMQFLPGTDFISSGYSAVPNYDNMFAGSNEDAEDFDDYNVLQRDLKVDGGLRPVLEADVVAIRNKAARALQAVFAGMGLPPITDEEVIAATYAHGSKDMPDRNIVEDIKFAQEIISKNRTGLEVVKALAQGGFEDVAQDMLNIQKAKIAGDYLHTSAIIKGDNQVLSAVNDVNDYAGPATGYRLEGARWEEIKNIPNALDPNELG

SEQ ID NO: 208 - protein, 554 aa, synthetic construct; identical to SEQ ID NO: 196

SEQ ID NO: 209 - protein, 370 aa, synthetic construct
MNTFSLQTRLYSGQGSLAVLKRFTNKHIWIICDGFLAHSPLLDTLRNALPADNRISVFSEITPDPTIHTVVQGIAQMQALQPQVVIGFGGGSAMDAAKAIVWFSQQSGINIETCVAIPTTSGTGSEVTSACVISDPDKGIKYPLFNNALYPDMAILDPELVVSVPPQITANTGMDVLTHALEAWVSPRASDFTDALAEKAAKLVFQYLPTAVEKGDCVATRGKMHNASTLAGMAFSQAGLGLNHAIAHQLGGQFHLPHGLANALLLTTVIRFNAGVPRAAKRYARLAKACGFCPAEANDIAAINALIQQIELLKQRCVLPSLAVALKEGRSDFSARIPAMVQAALADVTLRTNPRPANAEAIRELLEELL

SEQ ID NO: 210 - protein, 387 aa, synthetic construct
MSYRMFDYLVPNVNFFGPNAISVVGERCKLLGGKKALLVTDKGLRAIKDGAVDKTLTHLREAGIDVVVFDGVEPNPKDTNVRDGLEVFRKEHCDIIVTVGGGSPHDCGKGIGIAATHEGDLYSYAGIETLTNPLPPIVAVNTTAGTASEVTRHCVLTNTKTKVKFVIVSWRNLPSVSINDPLLMLGKPAPLTAATGMDALTHAVEAYISKDANPVTDAAAIQAIRLIARNLRQAVALGSNLKARENMAYASLLAGMAFNNANLGYVHAMAHQLGGLYDMPHGVANAVLLPHVARYNLIANPEKFADIAEFMGENTDGLSTMDAAELAIHAIARLSADIGIPQHLRDLGVKEADFPYMAEMALKDGNAFSNPRKGNEKEIAEIFRQAF

SEQ ID NO: 211 - protein, 471 aa, synthetic construct
MKQSTIALALLPLLFTPVTKARTPEMPVLENRAAQGDITAPGGARRLTGDQTAALRDSLSDKPAKNIILLIGDGMGDSEITAARNYAEGAGGFFKGIDALPLTGQYTHYALNKKTGKPDYVTDSAASATAWSTGVKTYNGALGVDIHEKDHPTILEMAKAAGLATGNVSTAELQDATPAALVAHVTSRKCYGPSATSEKCPGNALEKGGKGSITEQLLNARADVTLGGGAKTFAETATAGEWQGKTLREQAQARGYQLVSDAASLNSVTEANQQKPLLGLFADGNMPVRWLGPKATYHGNIDKPAVTCTPNPQRNDSVPTLAQMTDKAIELLSKNEKGFFLQVEGASIDKQDHAANPCGQIGETVDLDEAVQRALEFAKKEGNTLVIVTADHAHASQIVAPDTKAPGLTQALNTKDGAVMVMSYGNSEEDSQEHTGSQLRIAAYGPHAANVVGLTDQTDLFYTMKAALGLK

SEQ ID NO: 212 - protein, 546 aa, synthetic construct
MLTPKKWLLGVLVVSGMLGAQKTNAVPRPKLVVGLVVDQMRWDYLYRYYSKYGEGGFKRMLNTGYSLNNVHIDYVPTVTAIGHTSIFTGSVPSIHGIAGNDWYDKELGKSVYCTSDETVQPVGTTSNSVGQHSPRNLWSTTVTDQLGLATNFTSKVVGVSLKDRASILPAGHNPTGAFWFDDTTGKFITSTYYTKELPKWVNDFNNKNVPAQLVANGWNTLLPINQYTESSEDNVEWEGLLGSKKTPTFPYTDLAKDYEAKKGLIRTTPFGNTLTLQMADAAIDGNQMGVDDITDFLTVNLASTDYVGHNFGPNSIEVEDTYLRLDRDLADFFNNLDKKVGKGNYLVFLSADHGAAHSVGFMQAHKMPTGFFVEDMKKEMNAKLKQKFGADNIIAAAMNYQVYFDRKVLADSKLELDDVRDYVMTELKKEPSVLYVLSTDEIWESSIPEPIKSRVINGYNWKRSGDIQIISKDGYLSAYSKKGTTHSVWNSYDSHIPLLFMGWGIKQGESNQPYHMTDIAPTVSSLLKIQFPSGAVGKPITEVIGR

SEQ ID NO: 213 - protein, 237 aa, synthetic construct
MRKITQAISAVCLLFALNSSAVALASSPSPLNPGTNVARLAEQAPIHWVSVAQIENSLAGRPPMAVGFDIDDTVLFSSPGFWRGKKTFSPESEDYLKNPVFWEKMNNGWDEFSIPKEVARQLIDMHVRRGDAIFFVTGRSPTKTETVSKTLADNFHIPATNMNPVIFAGDKPGQNTKSQWLQDKNIRIFYGDSDNDITAARDVGARGIRILRASNSTYKPLPQAGAFGEEVIVNSEY

SEQ ID NO: 214 - protein, 203 aa, synthetic construct
MGVRNHRLLLLRHGETAWSTLGRHTGGTEVELTDTGRTQAELAGQLLGELELDDPIVICSPRRRTLDTAKLAGLTVNEVTGLLAEWDYGSYEGLTTPQIRESEPDWLVWTHGCPAGESVAQVNDRADSAVALALEHMSSRDVLFVSHGHFSRAVITRWVQLPLAEGSRFAMPTASIGICGFEHGVRQLAVLGLTGHPQPIAAG